European Patent Application EP 4 119 580 A1, published January 18, 2023. Title: ANTIBODIES AGAINST SIGNAL-REGULATORY PROTEIN ALPHA AND METHODS OF USE. Applicant: ALX Oncology Inc. Application Not Yet Assigned. The sequence listing filed with the application follows.

SEQUENCE LISTING (426 sequences)

SEQ ID NO: 1 - protein, 348 aa, Artificial Sequence
  Synthetic Construct
EEELQVIQPDKSVLVAAGETATLRCTATSLIPVGPIQWFRGAGPGRELIYNQKEGHFPRVTTVSDLTKRNNMDFSIRIGNITPADAGTYYCVKFRKGSPDDVEFKSGAGTELSVRAKPSESKYGPPCPPCPAPEFLGGPSVFLFPPKPKDTLMISRTPEVTCVVVDVSQEDPEVQFNWYVDGVEVHNAKTKPREEQFNSTYRVVSVLTVLHQDWLNGKEYKCKVSNKGLPSSIEKTISKAKGQPREPQVYTLPPSQEEMTKNQVSLTCLVKGFYPSDIAVEWESNGQPENNYKTTPPVLDSDGSFFLYSRLTVDKSRWQEGNVFSCSVMHEALHNHYTQKSLSLSLGK

SEQ ID NO: 2 - protein, 347 aa, Artificial Sequence
  Synthetic Construct
EEELQVIQPDKSVSVAAGESAILHCTVTSLIPVGPIQWFRGAGPARELIYNQKEGHFPRVTTVSESTKRENMDFSISISNITPADAGTYYCVKFRKGSPDTEFKSGAGTELSVRAKPSESKYGPPCPPCPAPEFLGGPSVFLFPPKPKDTLMISRTPEVTCVVVDVSQEDPEVQFNWYVDGVEVHNAKTKPREEQFNSTYRVVSVLTVLHQDWLNGKEYKCKVSNKGLPSSIEKTISKAKGQPREPQVYTLPPSQEEMTKNQVSLTCLVKGFYPSDIAVEWESNGQPENNYKTTPPVLDSDGSFFLYSRLTVDKSRWQEGNVFSCSVMHEALHNHYTQKSLSLSLGK

SEQ ID NO: 3 - protein, 346 aa, Artificial Sequence
  Synthetic Construct
KELKVTQPEKSVSVAAGDSTVLNCTLTSLLPVGPIKWYRGVGQSRLLIYSFTGEHFPRVTNVSDATKRNNMDFSIRISNVTPEDAGTYYCVKFQKGPSEPDTEIQSGGGTEVYVLAKPSDKTHTCPPCPAPEAAGAPSVFLFPPKPKDTLMISRTPEVTCVVVDVSHEDPEVKFNWYVDGVEVHNAKTKPREEQYASTYRVVSVLTVLHQDWLNGKEYKCKVSNKALPAPIEKTISKAKGQPREPQVYTLPPSREEMTKNQVSLTCLVKGFYPSDIAVEWESNGQPENNYKTTPPVLDSDGSFFLYSKLTVDKSRWQQGNVFSCSVMHEALHNHYTQKSLSLSPGK

SEQ ID NO: 4 - protein, 342 aa, Artificial Sequence
  Synthetic Construct
TEVKVIQPEKSVSVAAGDSTVLNCTLTSLLPVGPIRWYRGVGQSRQLIYSFTTEHFPRVTNVSDATKRSNLDFSIRISNVTPEDAGTYYCVKFQRGSPDTEIQSGGGTEVYVLAKDKTHTCPPCPAPEAAGAPSVFLFPPKPKDTLMISRTPEVTCVVVDVSHEDPEVKFNWYVDGVEVHNAKTKPREEQYASTYRVVSVLTVLHQDWLNGKEYKCKVSNKALPAPIEKTISKAKGQPREPQVYTLPPSREEMTKNQVSLTCLVKGFYPSDIAVEWESNGQPENNYKTTPPVLDSDGSFFLYSKLTVDKSRWQQGNVFSCSVMHEALHNHYTQKSLSLSPGK

SEQ ID NO: 5 - protein, 119 aa, Homo sapiens
EEELQVIQPDKSVLVAAGETATLRCTATSLIPVGPIQWFRGAGPGRELIYNQKEGHFPRVTTVSDLTKRNNMDFSIRIGNITPADAGTYYCVKFRKGSPDDVEFKSGAGTELSVRAKPS

SEQ ID NO: 6 - protein, 118 aa, Homo sapiens
EEELQVIQPDKSVSVAAGESAILHCTVTSLIPVGPIQWFRGAGPARELIYNQKEGHFPRVTTVSESTKRENMDFSISISNITPADAGTYYCVKFRKGSPDTEFKSGAGTELSVRAKPS

SEQ ID NO: 7 - protein, 119 aa, Mus musculus
KELKVTQPEKSVSVAAGDSTVLNCTLTSLLPVGPIKWYRGVGQSRLLIYSFTGEHFPRVTNVSDATKRNNMDFSIRISNVTPEDAGTYYCVKFQKGPSEPDTEIQSGGGTEVYVLAKPS

SEQ ID NO: 8 - protein, 115 aa, Mus musculus
TEVKVIQPEKSVSVAAGDSTVLNCTLTSLLPVGPIRWYRGVGQSRQLIYSFTTEHFPRVTNVSDATKRSNLDFSIRISNVTPEDAGTYYCVKFQRGSPDTEIQSGGGTEVYVLAK

SEQ ID NO: 9 - protein, 117 aa, Mus musculus
KELKVTQPEKSVSVAAGDSTVLNCTLTSLLPVGPIRWYRGVGPSRLLIYSFAGEYVPRIRNVSDTTKRNNMDFSIRISNVTPADAGIYYCVKFQKGSSEPDTEIQSGGGTEVYVLAK

SEQ ID NO: 10 - protein, 117 aa, Mus musculus
TEVKVTQPEKSVSVAAGDSTILNCTVTSLLPVGPIRWYRGVGQSRLLIYSFTGEHFPRIRNVSDTTKRNNMDFSIRISNVTPEDAGTYYCVKFQRGSSEPDTEIQSGGGTEVYVLAK

SEQ ID NO: 11 - protein, 118 aa, Macaca fascicularis
EEELQVIQPEKSVSVAAGESATLNCTATSLIPVGPIQWFRGVGPGRELIYHQKEGHFPRVTPVSDPTKRNNMDFSIRISNITPADAGTYYCVKFRKGSPDVELKSGAGTELSVRAKPS

SEQ ID NO: 12 - protein, 118 aa, Macaca fascicularis
EEELQVIQPEKSVSVAAGDSATLNCTVSSLIPVGPIQWFRGAGPGRELIYNLKEGHFPRVTAVSDPTKRNNMDFSIRISNITPADAGTYYCVKFRKGSPDVELKSGAGTELSVRAKPS

SEQ ID NO: 13 - protein, 119 aa, Homo sapiens
EDELQVIQPEKSVSVAAGESATLRCAMTSLIPVGPIMWFRGAGAGRELIYNQKEGHFPRVTTVSELTKRNNLDFSISISNITPADAGTYYCVKFRKGSPDDVEFKSGAGTELSVRAKPS

SEQ ID NO: 14 - protein, 119 aa, Homo sapiens
EEELQVIQPDKSISVAAGESATLHCTVTSLIPVGPIQWFRGAGPGRELIYNQKEGHFPRVTTVSDLTKRNNMDFSIRISNITPADAGTYYCVKFRKGSPDHVEFKSGAGTELSVRAKPS

SEQ ID NO: 15 - protein, 119 aa, Homo sapiens
EEELQMIQPEKLLLVTVGKTATLHCTVTSLLPVGPVLWFRGVGPGRELIYNQKEGHFPRVTTVSDLTKRNNMDFSIRISSITPADVGTYYCVKFRKGSPENVEFKSGPGTEMALGAKPS

SEQ ID NO: 16 - protein, 117 aa, Homo sapiens
QLLFNKTKSVEFTFSNDTVVIPCFVTNMEAQNTTEVYVKWKFKGRDIYTFDGALNKSTVPTDFSSAKIEVSQLLKGDASLKMDKSDAVSHTGNYTCEVTELTREGETIIELKYRVVS

SEQ ID NO: 17 - protein, 119 aa, Artificial Sequence
  Synthetic Construct
EEELQIIQPDKSVLVAAGETATLRCTITSLFPVGPIQWFRGAGPGRELIYNQREGPFPRVTTVSDTTKRNNMDFSIRIGAITPADAGTYYCVKFRKGSPDDVEFKSGAGTELSVRAKPS

SEQ ID NO: 18 - protein, 118 aa, Artificial Sequence
  Synthetic Construct
EEELQIIQPDKSVSVAAGESAILHCTITSLFPVGPIQWFRGAGPARVLIYNQRQGPFPRVTTVSETTKRENMDFSISISNITPADAGTYYCIKFRKGSPDTEFKSGAGTELSVRAKPS

SEQ ID NO: 19 - protein, 118 aa, Artificial Sequence
  Synthetic Construct
EEELQVIQPDKSVSVAAGESAILHCTVTSLFPVGPIQWFRGAGPARELIYNQRQGPFPRVTTVSESTKRENMDFSISISNITPADAGTYYCVKFRKGSPDTEFKSGAGTELSVRAKPS

SEQ ID NO: 20 - protein, 118 aa, Artificial Sequence
  Synthetic Construct
EEELQVIQPDKSVSVAAGESAILHCTITSLFPVGPIQWFRGAGPARVLIYNQRQGPFPRVTTVSETTKRENMDFSISISNITPADAGTYYCIKFRKGSPDTEFKSGAGTELSVRAKPS

SEQ ID NO: 21 - protein, 118 aa, Artificial Sequence
  Synthetic Construct
EEELQIIQPDKSVSVAAGESAILHCTVTSLFPVGPIQWFRGAGPARVLIYNQRQGPFPRVTTVSETTKRENMDFSISISNITPADAGTYYCIKFRKGSPDTEFKSGAGTELSVRAKPS

SEQ ID NO: 22 - protein, 118 aa, Artificial Sequence
  Synthetic Construct
EEELQIIQPDKSVSVAAGESAILHCTITSLIPVGPIQWFRGAGPARVLIYNQRQGPFPRVTTVSETTKRENMDFSISISNITPADAGTYYCIKFRKGSPDTEFKSGAGTELSVRAKPS

SEQ ID NO: 23 - protein, 118 aa, Artificial Sequence
  Synthetic Construct
EEELQIIQPDKSVSVAAGESAILHCTITSLFPVGPIQWFRGAGPARELIYNQRQGPFPRVTTVSETTKRENMDFSISISNITPADAGTYYCIKFRKGSPDTEFKSGAGTELSVRAKPS

SEQ ID NO: 24 - protein, 118 aa, Artificial Sequence
  Synthetic Construct
EEELQIIQPDKSVSVAAGESAILHCTITSLFPVGPIQWFRGAGPARVLIYNQKQGPFPRVTTVSETTKRENMDFSISISNITPADAGTYYCIKFRKGSPDTEFKSGAGTELSVRAKPS

SEQ ID NO: 25 - protein, 118 aa, Artificial Sequence
  Synthetic Construct
EEELQIIQPDKSVSVAAGESAILHCTITSLFPVGPIQWFRGAGPARVLIYNQREGPFPRVTTVSETTKRENMDFSISISNITPADAGTYYCIKFRKGSPDTEFKSGAGTELSVRAKPS

SEQ ID NO: 26 - protein, 118 aa, Artificial Sequence
  Synthetic Construct
EEELQIIQPDKSVSVAAGESAILHCTITSLFPVGPIQWFRGAGPARVLIYNQRQGHFPRVTTVSETTKRENMDFSISISNITPADAGTYYCIKFRKGSPDTEFKSGAGTELSVRAKPS

SEQ ID NO: 27 - protein, 118 aa, Artificial Sequence
  Synthetic Construct
EEELQIIQPDKSVSVAAGESAILHCTITSLFPVGPIQWFRGAGPARVLIYNQRQGPFPRVTTVSESTKRENMDFSISISNITPADAGTYYCIKFRKGSPDTEFKSGAGTELSVRAKPS

SEQ ID NO: 28 - protein, 118 aa, Artificial Sequence
  Synthetic Construct
EEELQIIQPDKSVSVAAGESAILHCTITSLFPVGPIQWFRGAGPARVLIYNQRQGPFPRVTTVSETTKRENMDFSISISNITPADAGTYYCVKFRKGSPDTEFKSGAGTELSVRAKPS

SEQ ID NO: 29 - protein, 118 aa, Artificial Sequence
  Synthetic Construct
EEELQVIQPDKSVSVAAGESAILHCTVTSLIPVGPIQWFRGAGPARELIYNQREGPFPRVTTVSESTKRENMDFSISISNITPADAGTYYCVKFRKGSPDTEFKSGAGTELSVRAKPS

SEQ ID NO: 30 - protein, 118 aa, Artificial Sequence
  Synthetic Construct
EEELQVIQPDKSVSVAAGESAILHCTVTSLFPVGPIQWFRGAGPARELIYNQREGPFPRVTTVSESTKRENMDFSISISNITPADAGTYYCVKFRKGSPDTEFKSGAGTELSVRAKPS

SEQ ID NO: 31 - protein, 118 aa, Artificial Sequence
  Synthetic Construct
EEELQVIQPDKSVSVAAGESAILHCTITSLFPVGPIQWFRGAGPARELIYNQREGPFPRVTTVSESTKRENMDFSISISNITPADAGTYYCVKFRKGSPDTEFKSGAGTELSVRAKPS

SEQ ID NO: 32 - protein, 118 aa, Artificial Sequence
  Synthetic Construct
EEELQVIQPDKSVSVAAGESAILHCTITSLFPVGPIQWFRGAGPARELIYNQREGPFPRVTTVSETTKRENMDFSISISNITPADAGTYYCVKFRKGSPDTEFKSGAGTELSVRAKPS

SEQ ID NO: 33 - protein, 118 aa, Artificial Sequence
  Synthetic Construct
EEELQIIQPDKSVSVAAGESAILHCTITSLFPVGPIQWFRGAGPARELIYNQREGPFPRVTTVSESTKRENMDFSISISNITPADAGTYYCVKFRKGSPDTEFKSGAGTELSVRAKPS

SEQ ID NO: 34 - protein, 118 aa, Artificial Sequence
  Synthetic Construct
EEELQVIQPDKSVSVAAGESAILHCTITSLIPVGPIQWFRGAGPARELIYNQREGPFPRVTTVSESTKRENMDFSISISNITPADAGTYYCVKFRKGSPDTEFKSGAGTELSVRAKPS

SEQ ID NO: 35 - protein, 118 aa, Artificial Sequence
  Synthetic Construct
EEELQIIQPDKSVSVAAGESAILHCTITSLFPVGPIQWFRGAGPARELIYNQREGPFPRVTTVSETTKRENMDFSISISNITPADAGTYYCVKFRKGSPDTEFKSGAGTELSVRAKPS

SEQ ID NO: 36 - protein, 119 aa, Artificial Sequence
  Synthetic Construct
EEELQVIQPDKSVLVAAGETATLRCTATSLFPVGPIQWFRGAGPGRELIYNQRQGPFPRVTTVSDLTKRNNMDFSIRIGNITPADAGTYYCVKFRKGSPDDVEFKSGAGTELSVRAKPS

SEQ ID NO: 37 - protein, 119 aa, Artificial Sequence
  Synthetic Construct
EEELQIIQPDKSVLVAAGETATLRCTITSLFPVGPIQWFRGAGPGRELIYNQREGPFPRVTTVSDLTKRNNMDFSIRIGNITPADAGTYYCVKFRKGSPDDVEFKSGAGTELSVRAKPS

SEQ ID NO: 38 - protein, 119 aa, Artificial Sequence
  Synthetic Construct
EEELQVIQPDKSVLVAAGETATLRCTITSLFPVGPIQWFRGAGPGRELIYNQREGPFPRVTTVSDTTKRNNMDFSIRIGNITPADAGTYYCVKFRKGSPDDVEFKSGAGTELSVRAKPS

SEQ ID NO: 39 - protein, 119 aa, Artificial Sequence
  Synthetic Construct
EEELQIIQPDKSVLVAAGETATLRCTITSLFPVGPIQWFRGAGPGRELIYNQREGPFPRVTTVSDTTKRNNMDFSIRIGNITPADAGTYYCVKFRKGSPDDVEFKSGAGTELSVRAKPS

SEQ ID NO: 40 - protein, 119 aa, Artificial Sequence
  Synthetic Construct
EEELQVIQPDKSVLVAAGETATLRCTITSLFPVGPIQWFRGAGPGRELIYNQREGPFPRVTTVSDLTKRNNMDFSIRIGNITPADAGTYYCVKFRKGSPDDVEFKSGAGTELSVRAKPS

SEQ ID NO: 41 - protein, 119 aa, Artificial Sequence
  Synthetic Construct
EEELQVIQPDKSVLVAAGETATLRCTATSLFPVGPIQWFRGAGPGRELIYNQREGPFPRVTTVSDLTKRNNMDFSIRIGNITPADAGTYYCVKFRKGSPDDVEFKSGAGTELSVRAKPS

SEQ ID NO: 42 - protein, 119 aa, Artificial Sequence
  Synthetic Construct
EEELQIIQPDKSVLVAAGETATLRCTITSLFPVGPIQWFRGAGPGRVLIYNQRQGPFPRVTTVSDTTKRNNMDFSIRIGNITPADAGTYYCIKFRKGSPDDVEFKSGAGTELSVRAKPS

SEQ ID NO: 43 - protein, 119 aa, Artificial Sequence
  Synthetic Construct
EEELQIIQPDKSVLVAAGETATLRCTITSLFPVGPIQWFRGAGPGRVLIYNQRQGPFPRVTTVSDTTKRNNMDFSIRIGAITPADAGTYYCIKFRKGSPDDVEFKSGAGTELSVRAKPS

SEQ ID NO: 44 - protein, 119 aa, Artificial Sequence
  Synthetic Construct
EEELQVIQPDKSVLVAAGETATLRCTATSLFPVGPIQWFRGAGPGRELIYNQRQGPFPRVTTVSDLTKRNNMDFSIRIGAITPADAGTYYCVKFRKGSPDDVEFKSGAGTELSVRAKPS

SEQ ID NO: 45 - protein, 119 aa, Artificial Sequence
  Synthetic Construct
EEELQIIQPDKSVLVAAGETATLRCTITSLFPVGPIQWFRGAGPGRVLIYNQREGPFPRVTTVSDTTKRNNMDFSIRIGAITPADAGTYYCIKFRKGSPDDVEFKSGAGTELSVRAKPS

SEQ ID NO: 46 - protein, 119 aa, Artificial Sequence
  Synthetic Construct
EEELQVIQPDKSVLVAAGETATLRCTATSLFPVGPIQWFRGAGPGRELIYNQREGPFPRVTTVSDLTKRNNMDFSIRIGAITPADAGTYYCVKFRKGSPDDVEFKSGAGTELSVRAKPS

SEQ ID NO: 47 - protein, 119 aa, Artificial Sequence
  Synthetic Construct
EEELQVIQPDKSVLVAAGETATLRCTITSLFPVGPIQWFRGAGPGRELIYNQREGPFPRVTTVSDLTKRNNMDFSIRIGAITPADAGTYYCVKFRKGSPDDVEFKSGAGTELSVRAKPS

SEQ ID NO: 48 - protein, 119 aa, Artificial Sequence
  Synthetic Construct
EEELQIIQPDKSVLVAAGETATLRCTITSLFPVGPIQWFRGAGPGRELIYNQREGPFPRVTTVSDLTKRNNMDFSIRIGAITPADAGTYYCVKFRKGSPDDVEFKSGAGTELSVRAKPS

SEQ ID NO: 49 - protein, 119 aa, Artificial Sequence
  Synthetic Construct
EEELQVIQPDKSVLVAAGETATLRCTITSLFPVGPIQWFRGAGPGRELIYNQREGPFPRVTTVSDTTKRNNMDFSIRIGAITPADAGTYYCVKFRKGSPDDVEFKSGAGTELSVRAKPS

SEQ ID NO: 50 - protein, 119 aa, Homo sapiens; identical to SEQ ID NO: 5

SEQ ID NO: 51 - protein, 119 aa, Artificial Sequence; identical to SEQ ID NO: 17
  Synthetic Construct

SEQ ID NO: 52 - protein, 119 aa, Artificial Sequence
  Synthetic Construct
EEELQVIQPDKSVLVAAGETATLRCTATSLFPVGPIQWFRGAGPGRELIYNQRQGPFPRVTTVSDLTKRNNMDFSIRIGNITVADAGTYYCVKFRKGSPDDVEFKSGAGTELSVRAKPS

SEQ ID NO: 53 - protein, 484 aa, Artificial Sequence
  Synthetic Construct
ALTQPASVSANPGETVEITCSGGGSNNAYGWFQQKSPGSAPLTVIYDNGKRPSDIPSRFSGSKSDSTGTLTITRVQAEDEAVYYCGSADNSGAGVFGAGTTLTVLGQSSRSSGGGGSSGGGGSMAAVTLDESGGGLQTPGGALSLVCKGSGFTFSSHAMNWVRQAPGKGLEWVAGISSDGRFTYYGAAVQGRATISRDNGQSTVRLQLNNLRAEDTATYYCTKNGGCGSGGDLDCIDAWGHGTEVIVSSSLDPKSSDKTHTCPPCPAPELLGGPSVFLFPPKPKDTLMISRTPEVTCVVVDVSHEDPEVKFNWYVDGVEVHNAKTKPREEQYNSTYRVVSVLTVLHQDWLNGKEYKCKVSNKALPAPIEKTISKAKGQPREPQVYTLPPSRDELTKNQVSLTCLVKGFYPSDIAVEWESNGQPENNYKTTPPVLDSDGSFFLYSKLTVDKSRWQQGNVFSCSVMHEALHNHYTQKSLSLSPGKV

SEQ ID NO: 54 - protein, 480 aa, Artificial Sequence
  Synthetic Construct
AVTQPASVSANPGETVRITCSGDSSSYYSWHQQKSPGSAPVSVIYSNTDRPSDIPSRFSGSASGSTATLTITGVQAEDEAVYFCGAYDSSSDSDIFGAGTTLTVLGQSSRSSGGGGSSGGGGSMAAVTLDESGGGLQTPGGGLSLVCKASGFDFSNFNMAWVRQGPGKGLEYVAEISDTGSTPYYGSAVQGRATISRDNGQSTVRLQLNNLRAEDTGTYFCTRNFGSSVSSIDAWGHGTEVIVSSSLDPKSSDKTHTCPPCPAPELLGGPSVFLFPPKPKDTLMISRTPEVTCVVVDVSHEDPEVKFNWYVDGVEVHNAKTKPREEQYNSTYRVVSVLTVLHQDWLNGKEYKCKVSNKALPAPIEKTISKAKGQPREPQVYTLPPSRDELTKNQVSLTCLVKGFYPSDIAVEWESNGQPENNYKTTPPVLDSDGSFFLYSKLTVDKSRWQQGNVFSCSVMHEALHNHYTQKSLSLSPGKV

SEQ ID NO: 55 - protein, 491 aa, Artificial Sequence
  Synthetic Construct
AVTQPSSVSANPGETVEITCSGSSTYYGWYQQKSPGSAPVTVIYDNDKRPSDIPSRFSGSKSGSTHTLIITGVQVEDEAVYFCGNEDNNYVAIFGAGTTLTVLGQSSRSSGGGGSSGGGGSMAAVTLDESGGGLQTPGGALSLVCKASGFTFSSYNMGWVRQAPGKGLEFVAGIYASGSSTDTDTTYGPAVAGRATISRDNGQSTVRLQLNNLRAEDTGTYYCAKAAGGCSTHTCTAYIADSIDAWGHGTEVIVSSSLDPKSSDKTHTCPPCPAPELLGGPSVFLFPPKPKDTLMISRTPEVTCVVVDVSHEDPEVKFNWYVDGVEVHNAKTKPREEQYNSTYRVVSVLTVLHQDWLNGKEYKCKVSNKALPAPIEKTISKAKGQPREPQVYTLPPSRDELTKNQVSLTCLVKGFYPSDIAVEWESNGQPENNYKTTPPVLDSDGSFFLYSKLTVDKSRWQQGNVFSCSVMHEALHNHYTQKSLSLSPGKV

SEQ ID NO: 56 - protein, 489 aa, Artificial Sequence
  Synthetic Construct
ALTQPSSVSANPGETVKITCSGDNSAHYYYGWYQQKSPGSAPVTVIYYNDKRPSGIPSRFSGSASGSTATLIITGVQVEDEAVYFCGSADSSNPAIFGAGTTLTVLGQSSRSSGGGGSSGGGGSMAAVTLDESGGGLQTPGRALSLVCRGSGFSISSYNMGWVRQAPGKGLEFIASIGSDGSSTHYAPAVKGRATITRDVGQSTVRLQLNNLRAEDTGTYFCAKDAYQCSYATCNDYLDTIDAWGHGTEVIVSSSLDPKSSDKTHTCPPCPAPELLGGPSVFLFPPKPKDTLMISRTPEVTCVVVDVSHEDPEVKFNWYVDGVEVHNAKTKPREEQYNSTYRVVSVLTVLHQDWLNGKEYKCKVSNKALPAPIEKTISKAKGQPREPQVYTLPPSRDELTKNQVSLTCLVKGFYPSDIAVEWESNGQPENNYKTTPPVLDSDGSFFLYSKLTVDKSRWQQGNVFSCSVMHEALHNHYTQKSLSLSPGKV

SEQ ID NO: 57 - protein, 487 aa, Artificial Sequence
  Synthetic Construct
AVTQPASVSANPGETVKITCSGSSSGSYGWYQQKSPGSAPVTLIYETNKRPSNIPSRFSGSKSGSTATLTITGVQADDEAVYYCGSEDSSTYLSIFGAGTTLTVLGQSSRSSGGGGSSGGGGSMAAVTLDESGGGLQTPGGALSLVCKASGFTFSSFNMGWVRQAPGKGLEFVAAIYSGNSAEYGAAVQGRATISRDNGQSTVRLQLNNLRAEDTGIYFCAKDAGSGCYSGVCAGTSSIDAWGHGTEVIVSSSLDPKSSDKTHTCPPCPAPELLGGPSVFLFPPKPKDTLMISRTPEVTCVVVDVSHEDPEVKFNWYVDGVEVHNAKTKPREEQYNSTYRVVSVLTVLHQDWLNGEEYKCKVSNKALPAPIEKTISKAKGQPREPQVYTLPPSRDELTKNQVSLTCLVKGFYPSDIAVEWESNGQPENNYKTTPPVLDSDGSFFLYSKLTVDKSRWQQGNVFSCSVMHEALHNHYTQKSLSLSPGKV

SEQ ID NO: 58 - protein, 489 aa, Artificial Sequence
  Synthetic Construct
AVTQPASVSANPGETVKITCSGDSSYYGWYQQKSPGSAPVTVIYDDNKRPSNIPSRFSGSKSGSTGTLTITGVQADDEAVYFCGNEDNSYVAIFGAGTTLTVLGQSSRSSGGGGSSGGGGSMAAVTLDESGGGLQTPGGALSLVCKASGFTFSSYNMGWVRQAPGKGLEFVAGIYIASGDLGTTYGAAVQGRATISRDDGQSTVRLQLNNLRAEDTGTYFCAKSAGGCSAHSCDTYIADSIDAWGHGTEVIVSSSLDPKSSDKTHTCPPCPAPELLGGPSVFLFPPKPKDTLMISRTPEVTCVVVDVSHEDPEVKFNWYVDGVEVHNAKTKPREEQYNSTYRVVSVLTVLHQDWLNGKEYKCKVSNKALPAPIEKTISKAKGQPREPQVYTLPPSRDELTKNQVSLTCLVKGFYPSDIAVEWESNGQPENNYKTTPPVLDSDGSFFLYSKLTVDKSRWQQGNVFSCSVMHEALHNHYTQKSLSLSPGKV

SEQ ID NO: 59 - protein, 490 aa, Artificial Sequence
  Synthetic Construct
AVTQPASVSANPGETVKITCSGSSSYYGWYRQKSPGSAPVTLIYDNDKRPSGIPSRFSGSKSGSTNTLTITGVQADDEAVYYCGNEDNSYVGIFGAGTTLTVLGQSSRSSGGGGSSGGGGSMAAVTLDESGGGLQTPGGALSLVCKASGFTFSSYNMGWVRQAPDKGLEFVAGIYTGSDAGLSTTYGAAVQGRATISRDNGQSTVRLQLNNLGAEDTGIYFCTKSAGGCSDYNCDAYIADSIDAWGHGTEVIVSSSLDPKSSDKTHTCPPCPAPELLGGPSVFLFPPKPKDTLMISRTPEVTCVVVDVSHEDPEVKFNWYVDGVEVHNAKTKPREEQYNSTYRVVSVLTVLHQDWLNGKEYKCKVSNKALPAPIEKTISKAKGQPREPQVYTLPPSRDELTKNQVSLTCLVKGFYPSDIAVEWESNGQPENNYKTTPPVLDSDGSFFLYSKLTVDKSRWQQGNVFSCSVMHEALHNHYTQKSLSLSPGKV

SEQ ID NO: 60 - protein, 489 aa, Artificial Sequence
  Synthetic Construct
AVTQPASVSANLGETVKITCSGDSSYYGWYQQKAPGSAPVTLIYDNDKRPSNIPSRFSGSKSGSTATLTITGVQADDEAVYYCGNEDMNYVGIFGAGTTLTVLGQSSRSSGGGGSSGGGGSMAAVTLDESGGGLQTPGGALSLVCKASGFTFNSYNMGWVRQAPGKGLEFVAGIYSAGGDTSTTYGAAVNGRATISRDNGQSTVRLQLNNLRAEDTGIYFCAKAAGGCTAHNCDAYIADSIDAWGHGTEVIVSSSLDPKSSDKTHTCPPCPAPELLGGPSVFLFPPKPKDTLMISRTPEVTCVVVDVSHEDPEVKFNWYVDGVEVHNAKTKPREEQYNSTYRVVSVLTVLHQDWLNGKEYKCKVSNKALPAPIEKTISKAKGQPREPQVYTLPPSRDELTKNQVSLTCLVKGFYPSDIAVEWESNGQPENNYKTTPPVLDSDGSFFLYSKLTVDKSRWQQGNVFSCSVMHEALHNHYTQKSLSLSPGKV

SEQ ID NO: 61 - protein, 480 aa, Artificial Sequence
  Synthetic Construct
ETVLTQSPATLSVSPGERATLSCRASQTVGSKLAWHQQKPGQAPRLLIYDATNRATGISDRFSGSGSGTDFTLTISSLQTEDSAVYYCQQYYYWPPYRFGGGTKVEIKGQSSRSSGGGGSSGGGGSDVQLVESGGGVVRPGESLRLSCAASGFSFSSYAMNWVRQAPGEGLEWVSRINSGGGGTDYAESVKGRFTISRDNSENTLYLQMNSLRAEDTAVYYCAKQYDWNSFFDYWGLGALVTVSSSLDPKSSDKTHTCPPCPAPELLGGPSVFLFPPKPKDTLMISRTPEVTCVVVDVSHEDPEVKFNWYVDGVEVHNAKTKPREEQYNSTYRVVSVLTVLHQDWLNGKEYKCKVSNKALPAPIEKTISKAKGQPREPQVYTLPPSRDELTKNQVSLTCLVKGFYPSDIAVEWESNGQPENNYKTTPPVLDSDGSFFLYSKLTVDKSRWQQGNVFSCSVMHEALHNHYTQKSLSLSPGKV

SEQ ID NO: 62 - protein, 480 aa, Artificial Sequence
  Synthetic Construct
ETVLTQSPATLSVSPGERATLSCRASQTVGSKLAWHQQKPGQAPRLLIYDATNRATGISDRFSGSRSGTDFTLTISSLQTEDSAVYYCQQYYYWPPYRFGGGTKVEIKGQSSRSSGGGGSSGGGGSDVQLVESGGGVVRPGESLRLSCAASGFSFSSYAMNWVRQAPGEGLEWVSRINSGGGGTDYAESVKGRFTISRDNSENTLYLQMNSLRAEDTAVYYCAKQYDWNSFFDYWGLGALVTVSSSLDPKSSDKTHTCPPCPAPELLGGPSVFLFPPKPKDTLMISRTPEVTCVVVDVSHEDPEVKFNWYVDGVEVHNAKTKPREEQYNSTYRVVSVLTVLHQDWLNGKEYKCKVSNKALPAPIEKTISKAKGQPREPQVYTLPPSRDELTKNQVSLTCLVKGFYPSDIAVEWESNGQPENNYKTTPPVLDSDGSFFLYSKLTVDKSRWQQGNVFSCSVMHEALHNHYTQKSLSLSPGKV

SEQ ID NO: 63 - protein, 480 aa, Artificial Sequence
  Synthetic Construct
ETVLTQSPATLSVSPGERATLSCRASQTVGSKLAWHQQKPGQAPRLLIYDATNRATGIPDRFSGSGSGTDFTLTISSLQTEDSAVYYCQQYYYWPPYRFGGGTKVEIKGQSSRSSGGGGSSRGGGSDVQLVESGGGVVRPGESLRLSCAASGFSFSSYAMNWVRQAPGEGLEWVSRINSGGGGTDYAESVKGRFTISRDNSENTLYLQMNSLRAEDTAVYYCAKQYDWNGFFDYWGLGALVTVSSSLDPKSSDKTHTCPPCPVPELLGGPSVFLFPPKPKDTLMISRTPEVTCVVVDVSHEDPEVKFNWYVDGVEVHNAKTKPREEQYNSTYRVVSVLTVLHQDWLNGKEYKCKVSNKALPAPIEKTISKAKGQPREPQVYTLPPSRDELTKNQVSLTCLVKGFYPSDIAVEWESNGQPENNYKTTPPVLDSDGSFFLYSKLTVDKSRWQQGNVFSCSVMHEALHNHYTQKSLSLSPGKV

SEQ ID NO: 64 - protein, 480 aa, Artificial Sequence
  Synthetic Construct
ETVLTQSPATLSVSPGERATLSCRASQTVGSKLAWHQQKPGQAPRLLIYDASRRATGIPDRFSGSGSGTDFTLTISSLQTEDSAVYYCQQYYYWPPYRFGGGTKVEIKGQSSRSSGGGGSSGGGGSDVQLVESGGGVVRPGESLRLSCAASGFSFSSYAMNWVRQAPGEGLEWVSRINSGGGGTDYAESVKGRFTISRDNSENTLYLQMNSLRAEDTAVYYCAKQYDWNGFFDYWGLGALVTVSSSLDPKSSDKTHTCPPCPAPELLGGPSVFLFPPKPKDTLMISRTPEVTCVVVDVSHEDPEVKFNWYVDGVEVHNAKTKPREEQYNSTYRVVSVLTVLHQDWLNGKEYKCKVSNKALPAPIEKTISKAKGQPREPQVYTLPPSRDELTKNQVSLTCLVKGFYPSDIAVEWESNGQPENNYKTTPPVLDSDGSFFLYSKLTVDKSRWQQGNVFSCSVMHEALHNHYTQKSLSLSPGKV

SEQ ID NO: 65 - protein, 481 aa, Artificial Sequence
  Synthetic Construct
EIVLTQSPATLSVSPGERATFSCRASQNVKNDLAWYQQRPGQAPRLLIYAARIRETGIPERFSGSGSGTEFTLTITSLQSEDFAVYYCQQYYDWPPFTFGGGTKVEIKGQSSRSSGGGGSSGGGGSDVQLLESGGGVVQPGGSLRLSCAASGFSFSNFAMTWVRQAPGEGLEWVSTIGSGDTYYADSVKGRFTISRDNSKNTLYLQMNSLRAEDTAVYYCAKDSTVSWSGDFFDYWGLGTLVTVSSSLDPKSSDKPHTCPPCPAPELLGGPSVFLFPPKPKDTLMISRTPEVTCVVVDVSHEDPEVKFNWYVDGVEVHNAKTKPREEQYNSTYRVVSVLTVLHQDWLNGKEYKCKVSNKALPAPIEKTISKAKGQPREPQVYTLPPSRDELTKNQVSLTCLVKGFYPSDIAVEWESNGQPENNYKTTPPVLDSDGSFFLYSKLTVDKSRWQQGNVFSCSVMHEALHNHYTQKSLSLSPGKV

SEQ ID NO: 66 - protein, 481 aa, Artificial Sequence
  Synthetic Construct
EIVLTQSPATLSVSPGERATFSCRASQNVKNDLAWYQQRPGQAPRLLIYAARIRETGIPERFSGSGSGTEFTLTITSLQSEDFAVYYCQQYYDWPPFTFGGGTKVEIKGQSSRSSGGGGSSGGGGSDVQLVESGGGVVQPGGSLRLSCAASGFSFSNFAMTWVRQAPGEGLEWVSTIGSGDTYYADSVKGRFTISRDNSKNTLYLQMNSLRAEDTAVYYCAKDSTVSWSGDFFDYWGLGTRVTVSSSLDPKSSDKTHTCPPCPAPELLGGPSVFLFPPKPKDTLMISRTPEVTCVVVDVSHEDPEVKFNWYVDGVEVHNAKTKPREEQYNSTYRVVSVLTVLHQDWLNGKEYKCKVSNKALPAPIEKTISKAKGQPREPQVYTLPPSRDELTKNQVSLTCLVKGFYPSDIAVEWESNGQPENNYKTTPPVLDSDGSFFLYSKLTVDKSRWQQGNVFSCSVMHEALHNHYTQKSLSLSPGKV

SEQ ID NO: 67 - protein, 481 aa, Artificial Sequence
  Synthetic Construct
EIVLTQSPATLSVSPGERATFSCRASQNVKNDLAWYQQRPGQAPRLLIYAARIRETGIPERFSGSGSGTEFTLTITSLQSEDFAVYYCQQYYDWPPFTFGGGTKVEIKGQSSRSSGGGGSSGGGGSDVQLVESGGGVVRPGESLRLSCAASGFRFSNFAMTWVRQAPGEGLEWVSTIGSGDTYYADSVKGRFTISRDNSKNTLYLQMNSLRAEDTAVYYCAKDSTVSWSGDFFDYWGLGTLVTVSSSLDPKSSDKTHTCPPCPAPELLGGPSVFLFPPKPKDTLMISRTPEVTCVVVDVSHEDPEVKFNWYVDGVEVHNAKTKPREEQYNSTYRVVSVLTVLHQDWLNGKEYKCKVSNKALPAPIEKTISKAKGQPREPQVYTLPPSRDELTKNQVSLTCLVKGFYPSDIAVEWESNGQPENNYKTTPPVLDSDGSFFLYSKLTVDKSRWQQGNVFSCSVMHEALHNHYTQKSLSLSPGKV

SEQ ID NO: 68 - protein, 478 aa, Artificial Sequence
  Synthetic Construct
EIVLTQSPGTLSVSPGERVTLTCRASQGIAGKIAWYQQKPGQAPRLLIYDASSRATGIPGRFSGSGSGTEFTLTITSLQSEDFAVYYCQQHYDWSPLTFGGGTKVEIKGQSSRSSGGGGSSGGGGSDVQLVESGGGLVQPGGSLRLSCTASGFTFRNYGMSWVRQAPGEGLEWVSASSGSGSTYYTDSVKGRFTISRDNSKNTLYLQMNSLRAEDTAIYYCAKVTWNNFFDYWGLGTLVTVSSSLDPKSSDKTHTCPPCPAPELLGGPSVFLFPPKPKDTLMISRTPEVTCVVVDVSHEDPEVKFNWYVDGVEVHNAKTKPREEQYNSTYRVVSVLTVLHQDWLNGKEYKCKVSNKALPAPIEKTISKAKGQPREPQVYTLPPSRDELTKNQVSLTCLVKGFYPSDIAVEWESNGQPENNYKTTPPVLDSDGSFFLYSKLTVDKSRWQQGNVFSCSVMHEALHNHYTQKSLSLSPGKV

SEQ ID NO: 69 - protein, 478 aa, Artificial Sequence
  Synthetic Construct
EIVLTQSPGTLTLSPGERATLSCRASQSIGSSYLAWYQQKPGQAPRLLIYDATNRATGIPDRFSGSGSGTDFTLTISSLQTEDSAVYYCQQYYYWPPYRFGGGTKVEIKGQSSRSSGGGSSSGGGGSDVQLVESGGGVVRPGESLRLSCAASGFTFSNYDMTWVRQAPGEGLEWVSGISGNGGSTYYADSVKGRFTISRDNSKNTLYLQMNSLRAEDTAVYYCAMNRWWFDYWGLGTLVTVSSSLDPKSSDKTHTCPPCPAPELLGGPSVFLFPPKPKDTLMISRTPEVTCVVVDVSHEDPEVKFNWYVDGVEVHNAKTKPREEQYNSTYRVVSVLTVLHQDWLNGKEYKCKVSNKALPAPIEKTISKAKGQPREPQVYTLPPSRDELTKNQVSLTCLVKGFYPSDIAVEWESNGQPENNYKTTPPVLDSDGSFFLYSKLTVDKSRWQQGNVFSCSVMHEALHNHYTQKSLSLSPGKV

SEQ ID NO: 70 - protein, 480 aa, Artificial Sequence
  Synthetic Construct
ETVLTQSPATLSVSPGERATLSCRASQTVGSKLAWHQQKPGQAPRLLIYDASNRATGIPDRFSGSGSGTDFTLTISSLQTEDSAVYYCQQYYYWPPYRFGGGTKVEIKGQSSRSSGGGGSSGGGGSDVQLVESGGGVVRPGESLRLSCAASGFSFRSYAMNWVRQAPGEGLEWVSRIDSGGGGTDYADSVKGRFTISRDNSKNTLYLQMNSLRAEDTAVYYCAKQYDWNSFFDYWGLGAPVTVSSSLDPKSSDKTHTCPPCPAPELLGGPSVFLFPPKPKDTLMISRTPEVTCVVVDVSHEDPEVKFNWYVDGVEVHNAKTKPREEQYNSTYRVVSVLTVLHQDWLNGKEYKCKVSNKALPAPIEKTISKAKGQPREPQVYTLPPSRDELTKNQVSLTCLVKGFYPSDIAVEWESNGQPENNYKTTPPVLDSDGSFFLYSKLTVDKSRWQQGNVFSCSVMHEALHNHYTQKSLSLSPGKV

SEQ ID NO: 71 - protein, 483 aa, Artificial Sequence
  Synthetic Construct
EIVLTQSPGTLSVSPGERATLSCRASQNVRSDLAWYQQKLGQAPRLLIYDANTRATDIPDRFSGSGSGTEFTLTISSLQSEDFAVYYCQHYYDWPPVTFGGGTKVEIKGQSSRSSGGGGSSGGGGSDVQLVESGGGVVRPGESLRLSCAASGFTFSNYAMSWVRQAPGEGLEWVSLITTNGDGAYYADSVKGRFTISRDNSKNTLYLQMNSLRAEDTAIYYCAKDGAAHYYDIFFDYWGLGTPVTVSSSLDPKSSDKTHTCPPCPAPELLGGPSVFLFPPKPKDTLMISRTPEVTCVVVDVSHEDPEVKFNWYVDGVEVHNAKTKPREEQYNSTYRVVSVLTVLHQDWLNGKEYKCKVSNKALPAPIEKTISKAKGQPREPQVYTLPPSRDELTKNQVSLTCLVKGFYPSDIAVEWESNGQPENNYKTTPPVLDSDGSFFLYSKLTVDKSRWQQGNVFSCSVMHEALHNHYTQKSLSLSPGKV

SEQ ID NO: 72 - protein, 481 aa, Artificial Sequence
  Synthetic Construct
EIVLTQSPATLSVSPGERVTFSCRASQNVRSDIAWYQQKPGQAPRLLIYAASSRDTGIPDRFSGSGSGTDFTLTISSLQSEDFGVYYCQQYYDWPPFTFGGGTKVEIKGQSSRSSGGGGSSGGGGSDVQLVESGGGVVRPGESLRLSCAASGFSFSIYAMSWVRQAPGEGLEWVSTIGADDTYYADSVKGRFTISRDNSKNTLYLQMNSLRAEDTAVYYCAKDSTVGWSGDFFDYWGLGTLVTVSSSLDPKSSDKTHTCPPCPAPELLGGPSVFLFPPKPKDTLMISRTPEVTCVVVDVSHEDPEVKFNWYVDGVEVHNAKTKPREEQYNSTYRVVSVLTVLHQDWLNGKEYKCKVSNKALPAPIEKTISKAKGQPREPQVYTLPPSRDELTKNQVSLTCLVKGFYPSDIAVEWESNGQPENNYKTTPPVLDSDGSFFLYSKLTVDKSRWQQGNVFSCSVMHEALHNHYTQKSLSLSPGKV

SEQ ID NO: 73 - protein, 480 aa, Artificial Sequence
  Synthetic Construct
ETVLTQSPGTLTLSPGERATLTCRASQSVYTYLAWYQEKPGQAPRLLIYGASSRATGIPDRFSGSGSGTVFTLTISSLQSEDFAVYYCQQYYDRPPLTFGGGTKVEIKGQSSRSSGGGGSSGGGGSDVQLVESGGGVVRPGESLRLSCAASGFTFSSYDMNWVRQAPGEGLEWVSLISGSGEIIYYADSVKGRFTISRDNSKNTLYLQMNSLRAEDTAVYYCAKENNRYRFFDDWGLGTLVTVSSSLDPKSSDKTHTCPPCPAPELLGGPSVFLFPPKPKDTLMISRTPEVTCVVVDVSHEDPEVKFNWYVDGVEVHNAKTKPREEQYNSTYRVVSVLTVLHQDWLNGKEYKCKVSNKALPAPIEKTISKAKGQPREPQVYTLPPSRDELTKNQVSLTCLVKGFYPSDIAVEWESNGQPENNYKTTPPVLDSDGSFFLYSKLTVDKSRWQQGNVFSCSVMHEALHNHYTQKSLSLSPGKV

SEQ ID NO: 74 - protein, 315 aa, Artificial Sequence
  Synthetic Construct
EIVLTQSPGTLSVSPGERVILTCRASQSVDTYNLAWYQQKPGQAPRLLIYDLSTRATGIPDRFSGSGSGTEFTLTINSLEPEDFAVYYCHQYYDWPPYTFGGGTKVEIKGQSSRSSGGGGSSGGGGSDVQLVESGGGVVRPGESLRLSCAASGFTFSNYAMNWVRQAPGEGLEWVSGISGRGGDTYYADSVKGRFTISRDNSKNTLYLQMNSLRAEDTAIYYCAKGTWNYGSFDYWGLGTLVTVSSSLDPKSSDKTDTCPPCPAPELLGGPSVFLFPPKPKDTLMISRTPEVTCVVVDVSHEDPEVKFNWYVDGV

SEQ ID NO: 75 - protein, 481 aa, Artificial Sequence
  Synthetic Construct
EIVLTQSPATLSVSPGERATFSCRASQNVKNDLAWYQQRPGQAPRLLIYAARIRETGIPERFSGSGSGTEFTLTITSLQSEDFAVYYCQQYYDWPPFTFGGGTKVEIKGQSSRSSGGGGSSGGGGSDVQLVESGGGVVQPGGSLRLSCAASGFSFSNFAMTWVRQAPGEGLEWVSTIGSGDTYYADSVKGRFTISRDNSKNTLYLQMNSLRAEDTAVYYCAKDSTVSWSGDFFDYWGLGTLVTVSSSLDPKSSDKTHTCPPCPAPELLGGPSVFLFPPKPKDTLMISRTPEVTCVVVDVSHEDPEVKFNWYVDGVEVHNAKTKPREEQYNSTYRVVSVLTVLHQDWLNGKEYKCKVSNKALPAPIEKTISKAKGQPREPQVYTLPPSRDELTKNQVSLTCLVKGFYPSDIAVEWESNGQPENNYKTTPPVLDSDGSFFLYSKLTVDKSRWQQGNVFSCSVMHEALHNHYTQKSLSLSPGKV

SEQ ID NO: 76 - protein, 118 aa, Homo sapiens
EEELQVIQPDKSVSVAAGESAILLCTVTSLIPVGPIQWFRGAGPARELIYNQKEGHFPRVTTVSESTKRENMDFSISISNITPADAGTYYCVKFRKGSPDTEFKSGAGTELSVRAKPS

SEQ ID NO: 77 - protein, 119 aa, Homo sapiens
EEGLQVIQPDKSVSVAAGESAILHCTATSLIPVGPIQWFRGAGPGRELIYNQKEGHFPRVTTVSDLTKRNNMDFSIRIGNITPADAGTYYCVKFRKGSPDDVEFKSGAGTELSVRAKPS

SEQ ID NO: 78 - protein, 119 aa, Homo sapiens
EEELQVIQPDKFVLVAAGETATLRCTATSLIPVGPIQWFRGAGPGRELIYNQKEGHFPRVTTVSDLTKRNNMDFSIRIGNITPADAGTYYCVKFRKGSPDDVEFKSGAGTELSVRAKPS

SEQ ID NO: 79 - protein, 119 aa, Homo sapiens
EEELQVIQPDKSVLVAAGETATLRCTATSLIPVGPIQWFRGAGPGRELIYNQKEGHFPRVTTVSDLTKRNNMDFPIRIGNITPADAGTYYCVKFRKGSPDDVEFKSGAGTELSVRAKPS

SEQ ID NO: 80 - protein, 118 aa, Homo sapiens
EEELQVIQPDKSVSVAAGESAILHCTVTSLIPVGPIQWFRGAGPARELIYNQKEGHFPRVTTVSESTKRENMDFSISISNITPADAGTYYCVKFRKGSPDTEFKSGAGTELSVRGKPS

SEQ ID NO: 81 - protein, 118 aa, Homo sapiens
EEELQVIQPDKSVLVAAGETATLRCTATSLIPVGPIQWFRGAGPARELIYNQKEGHFPRVTTVSESTKRENMDFSISISNITPADAGTYYCVKFRKGSPDTEFKSGAGTELSVRAKPS

SEQ ID NO: 82 - protein, 119 aa, Homo sapiens
EEELQVIQPDKSVLVAAGETATLRCTATSLIPVGPIQWFRGAGPGRELIYNQKEGHFPRVTTVSDLTKRNNMDFSIRISNITPADAGTYYCVKFRKGSPDDVEFKSGAGTELSVRAKPS

SEQ ID NO: 83 - protein, 118 aa, Homo sapiens; identical to SEQ ID NO: 6

SEQ ID NO: 84 - protein, 110 aa, Gallus gallus
DFKLQQPQSSVVVIKGDTLTLNCTASGSGPIGAVKWVKGWGSDNQTVYEHKGSFPRVMRAVPDPTNDFTIRISNVSLEDAGTYYCVKLRKGIVDDVVFTRGGGTEVSVHA

SEQ ID NO: 85 - protein, 105 aa, Artificial Sequence
  Synthetic Construct
ALTQPASVSANPGETVEITCSGGGSNNAYGWFQQKSPGSAPLTVIYDNGKRPSDIPSRFSGSKSDSTGTLTITRVQAEDEAVYYCGSADNSGAGVFGAGTTLTVL

SEQ ID NO: 86 - protein, 105 aa, Artificial Sequence
  Synthetic Construct
AVTQPASVSANPGETVRITCSGDSSSYYSWHQQKSPGSAPVSVIYSNTDRPSDIPSRFSGSASGSTATLTITGVQAEDEAVYFCGAYDSSSDSDIFGAGTTLTVL

SEQ ID NO: 87 - protein, 103 aa, Artificial Sequence
  Synthetic Construct
AVTQPSSVSANPGETVEITCSGSSTYYGWYQQKSPGSAPVTVIYDNDKRPSDIPSRFSGSKSGSTHTLIITGVQVEDEAVYFCGNEDNNYVAIFGAGTTLTVL

SEQ ID NO: 88 - protein, 106 aa, Artificial Sequence
  Synthetic Construct
ALTQPSSVSANPGETVKITCSGDNSAHYYYGWYQQKSPGSAPVTVIYYNDKRPSGIPSRFSGSASGSTATLIITGVQVEDEAVYFCGSADSSNPAIFGAGTTLTVL

SEQ ID NO: 89 - protein, 105 aa, Artificial Sequence
  Synthetic Construct
AVTQPASVSANPGETVKITCSGSSSGSYGWYQQKSPGSAPVTLIYETNKRPSNIPSRFSGSKSGSTATLTITGVQADDEAVYYCGSEDSSTYLSIFGAGTTLTVL

SEQ ID NO: 90 - protein, 103 aa, Artificial Sequence
  Synthetic Construct
AVTQPASVSANPGETVKITCSGDSSYYGWYQQKSPGSAPVTVIYDDNKRPSNIPSRFSGSKSGSTGTLTITGVQADDEAVYFCGNEDNSYVAIFGAGTTLTVL

SEQ ID NO: 91 - protein, 103 aa, Artificial Sequence
  Synthetic Construct
AVTQPASVSANPGETVKITCSGSSSYYGWYRQKSPGSAPVTLIYDNDKRPSGIPSRFSGSKSGSTNTLTITGVQADDEAVYYCGNEDNSYVGIFGAGTTLTVL

SEQ ID NO: 92 - protein, 103 aa, Artificial Sequence
  Synthetic Construct
AVTQPASVSANLGETVKITCSGDSSYYGWYQQKAPGSAPVTLIYDNDKRPSNIPSRFSGSKSGSTATLTITGVQADDEAVYYCGNEDMNYVGIFGAGTTLTVL

SEQ ID NO: 93 - protein, 108 aa, Artificial Sequence
  Synthetic Construct
ETVLTQSPATLSVSPGERATLSCRASQTVGSKLAWHQQKPGQAPRLLIYDATNRATGISDRFSGSGSGTDFTLTISSLQTEDSAVYYCQQYYYWPPYRFGGGTKVEIK

SEQ ID NO: 94 - protein, 108 aa, Artificial Sequence
  Synthetic Construct
ETVLTQSPATLSVSPGERATLSCRASQTVGSKLAWHQQKPGQAPRLLIYDATNRATGISDRFSGSRSGTDFTLTISSLQTEDSAVYYCQQYYYWPPYRFGGGTKVEIK

SEQ ID NO: 95 - protein, 108 aa, Artificial Sequence
  Synthetic Construct
ETVLTQSPATLSVSPGERATLSCRASQTVGSKLAWHQQKPGQAPRLLIYDATNRATGIPDRFSGSGSGTDFTLTISSLQTEDSAVYYCQQYYYWPPYRFGGGTKVEIK

SEQ ID NO: 96 - protein, 108 aa, Artificial Sequence
  Synthetic Construct
ETVLTQSPATLSVSPGERATLSCRASQTVGSKLAWHQQKPGQAPRLLIYDASRRATGIPDRFSGSGSGTDFTLTISSLQTEDSAVYYCQQYYYWPPYRFGGGTKVEIK

SEQ ID NO: 97 - protein, 108 aa, Artificial Sequence
  Synthetic Construct
EIVLTQSPATLSVSPGERATFSCRASQNVKNDLAWYQQRPGQAPRLLIYAARIRETGIPERFSGSGSGTEFTLTITSLQSEDFAVYYCQQYYDWPPFTFGGGTKVEIK

SEQ ID NO: 98 - protein, 108 aa, Artificial Sequence; identical to SEQ ID NO: 97
  Synthetic Construct

SEQ ID NO: 99 - protein, 108 aa, Artificial Sequence; identical to SEQ ID NO: 97
  Synthetic Construct

SEQ ID NO: 100 - protein, 108 aa, Artificial Sequence
  Synthetic Construct
EIVLTQSPGTLSVSPGERVTLTCRASQGIAGKIAWYQQKPGQAPRLLIYDASSRATGIPGRFSGSGSGTEFTLTITSLQSEDFAVYYCQQHYDWSPLTFGGGTKVEIK

SEQ ID NO: 101 - protein, 109 aa, Artificial Sequence
  Synthetic Construct
EIVLTQSPGTLTLSPGERATLSCRASQSIGSSYLAWYQQKPGQAPRLLIYDATNRATGIPDRFSGSGSGTDFTLTISSLQTEDSAVYYCQQYYYWPPYRFGGGTKVEIK

SEQ ID NO: 102 - protein, 108 aa, Artificial Sequence
  Synthetic Construct
ETVLTQSPATLSVSPGERATLSCRASQTVGSKLAWHQQKPGQAPRLLIYDASNRATGIPDRFSGSGSGTDFTLTISSLQTEDSAVYYCQQYYYWPPYRFGGGTKVEIK

SEQ ID NO: 103 - protein, 108 aa, Artificial Sequence
  Synthetic Construct
EIVLTQSPGTLSVSPGERATLSCRASQNVRSDLAWYQQKLGQAPRLLIYDANTRATDIPDRFSGSGSGTEFTLTISSLQSEDFAVYYCQHYYDWPPVTFGGGTKVEIK

SEQ ID NO: 104 - protein, 108 aa, Artificial Sequence
  Synthetic Construct
EIVLTQSPATLSVSPGERVTFSCRASQNVRSDIAWYQQKPGQAPRLLIYAASSRDTGIPDRFSGSGSGTDFTLTISSLQSEDFGVYYCQQYYDWPPFTFGGGTKVEIK

SEQ ID NO: 105 - protein, 108 aa, Artificial Sequence
  Synthetic Construct
ETVLTQSPGTLTLSPGERATLTCRASQSVYTYLAWYQEKPGQAPRLLIYGASSRATGIPDRFSGSGSGTVFTLTISSLQSEDFAVYYCQQYYDRPPLTFGGGTKVEIK

SEQ ID NO: 106 - protein, 109 aa, Artificial Sequence
  Synthetic Construct
EIVLTQSPGTLSVSPGERVILTCRASQSVDTYNLAWYQQKPGQAPRLLIYDLSTRATGIPDRFSGSGSGTEFTLTINSLEPEDFAVYYCHQYYDWPPYTFGGGTKVEIK

SEQ ID NO: 107 - protein, 108 aa, Artificial Sequence; identical to SEQ ID NO: 97
  Synthetic Construct

SEQ ID NO: 108 - protein, 124 aa, Artificial Sequence
  Synthetic Construct
AVTLDESGGGLQTPGGALSLVCKGSGFTFSSHAMNWVRQAPGKGLEWVAGISSDGRFTYYGAAVQGRATISRDNGQSTVRLQLNNLRAEDTATYYCTKNGGCGSGGDLDCIDAWGHGTEVIVSS

SEQ ID NO: 109 - protein, 120 aa, Artificial Sequence
  Synthetic Construct
AVTLDESGGGLQTPGGGLSLVCKASGFDFSNFNMAWVRQGPGKGLEYVAEISDTGSTPYYGSAVQGRATISRDNGQSTVRLQLNNLRAEDTGTYFCTRNFGSSVSSIDAWGHGTEVIVSS

SEQ ID NO: 110 - protein, 133 aa, Artificial Sequence
  Synthetic Construct
AVTLDESGGGLQTPGGALSLVCKASGFTFSSYNMGWVRQAPGKGLEFVAGIYASGSSTDTDTTYGPAVAGRATISRDNGQSTVRLQLNNLRAEDTGTYYCAKAAGGCSTHTCTAYIADSIDAWGHGTEVIVSS

SEQ ID NO: 111 - protein, 128 aa, Artificial Sequence
  Synthetic Construct
AVTLDESGGGLQTPGRALSLVCRGSGFSISSYNMGWVRQAPGKGLEFIASIGSDGSSTHYAPAVKGRATITRDVGQSTVRLQLNNLRAEDTGTYFCAKDAYQCSYATCNDYLDTIDAWGHGTEVIVSS

SEQ ID NO: 112 - protein, 127 aa, Artificial Sequence
  Synthetic Construct
AVTLDESGGGLQTPGGALSLVCKASGFTFSSFNMGWVRQAPGKGLEFVAAIYSGNSAEYGAAVQGRATISRDNGQSTVRLQLNNLRAEDTGIYFCAKDAGSGCYSGVCAGTSSIDAWGHGTEVIVSS

SEQ ID NO: 113 - protein, 131 aa, Artificial Sequence
  Synthetic Construct
AVTLDESGGGLQTPGGALSLVCKASGFTFSSYNMGWVRQAPGKGLEFVAGIYIASGDLGTTYGAAVQGRATISRDDGQSTVRLQLNNLRAEDTGTYFCAKSAGGCSAHSCDTYIADSIDAWGHGTEVIVSS

SEQ ID NO: 114 - protein, 132 aa, Artificial Sequence
  Synthetic Construct
AVTLDESGGGLQTPGGALSLVCKASGFTFSSYNMGWVRQAPDKGLEFVAGIYTGSDAGLSTTYGAAVQGRATISRDNGQSTVRLQLNNLGAEDTGIYFCTKSAGGCSDYNCDAYIADSIDAWGHGTEVIVSS

SEQ ID NO: 115 - protein, 131 aa, Artificial Sequence
  Synthetic Construct
AVTLDESGGGLQTPGGALSLVCKASGFTFNSYNMGWVRQAPGKGLEFVAGIYSAGGDTSTTYGAAVNGRATISRDNGQSTVRLQLNNLRAEDTGIYFCAKAAGGCTAHNCDAYIADSIDAWGHGTEVIVSS

SEQ ID NO: 116 - protein, 118 aa, Artificial Sequence
  Synthetic Construct
VQLVESGGGVVRPGESLRLSCAASGFSFSSYAMNWVRQAPGEGLEWVSRINSGGGGTDYAESVKGRFTISRDNSENTLYLQMNSLRAEDTAVYYCAKQYDWNSFFDYWGLGALVTVSS

SEQ ID NO: 117 - protein, 118 aa, Artificial Sequence; identical to SEQ ID NO: 116
  Synthetic Construct

SEQ ID NO: 118 - protein, 118 aa, Artificial Sequence
  Synthetic Construct
VQLVESGGGVVRPGESLRLSCAASGFSFSSYAMNWVRQAPGEGLEWVSRINSGGGGTDYAESVKGRFTISRDNSENTLYLQMNSLRAEDTAVYYCAKQYDWNGFFDYWGLGALVTVSS

SEQ ID NO: 119 - protein, 118 aa, Artificial Sequence; identical to SEQ ID NO: 118
  Synthetic Construct

SEQ ID NO: 120 - protein, 119 aa, Artificial Sequence
  Synthetic Construct
VQLLESGGGVVQPGGSLRLSCAASGFSFSNFAMTWVRQAPGEGLEWVSTIGSGDTYYADSVKGRFTISRDNSKNTLYLQMNSLRAEDTAVYYCAKDSTVSWSGDFFDYWGLGTLVTVSS

SEQ ID NO: 121 - protein, 119 aa, Artificial Sequence
  Synthetic Construct
VQLVESGGGVVQPGGSLRLSCAASGFSFSNFAMTWVRQAPGEGLEWVSTIGSGDTYYADSVKGRFTISRDNSKNTLYLQMNSLRAEDTAVYYCAKDSTVSWSGDFFDYWGLGTRVTVSS

SEQ ID NO: 122 - protein, 119 aa, Artificial Sequence
  Synthetic Construct
VQLVESGGGVVRPGESLRLSCAASGFRFSNFAMTWVRQAPGEGLEWVSTIGSGDTYYADSVKGRFTISRDNSKNTLYLQMNSLRAEDTAVYYCAKDSTVSWSGDFFDYWGLGTLVTVSS

SEQ ID NO: 123 - protein, 116 aa, Artificial Sequence
  Synthetic Construct
VQLVESGGGLVQPGGSLRLSCTASGFTFRNYGMSWVRQAPGEGLEWVSASSGSGSTYYTDSVKGRFTISRDNSKNTLYLQMNSLRAEDTAIYYCAKVTWNNFFDYWGLGTLVTVSS

SEQ ID NO: 124 - protein, 115 aa, Artificial Sequence
  Synthetic Construct
VQLVESGGGVVRPGESLRLSCAASGFTFSNYDMTWVRQAPGEGLEWVSGISGNGGSTYYADSVKGRFTISRDNSKNTLYLQMNSLRAEDTAVYYCAMNRWWFDYWGLGTLVTVSS

SEQ ID NO: 125 - protein, 118 aa, Artificial Sequence
  Synthetic Construct
VQLVESGGGVVRPGESLRLSCAASGFSFRSYAMNWVRQAPGEGLEWVSRIDSGGGGTDYADSVKGRFTISRDNSKNTLYLQMNSLRAEDTAVYYCAKQYDWNSFFDYWGLGAPVTVSS

SEQ ID NO: 126 - protein, 121 aa, Artificial Sequence
  Synthetic Construct
VQLVESGGGVVRPGESLRLSCAASGFTFSNYAMSWVRQAPGEGLEWVSLITTNGDGAYYADSVKGRFTISRDNSKNTLYLQMNSLRAEDTAIYYCAKDGAAHYYDIFFDYWGLGTPVTVSS

SEQ ID NO: 127 - protein, 119 aa, Artificial Sequence
  Synthetic Construct
VQLVESGGGVVRPGESLRLSCAASGFSFSIYAMSWVRQAPGEGLEWVSTIGADDTYYADSVKGRFTISRDNSKNTLYLQMNSLRAEDTAVYYCAKDSTVGWSGDFFDYWGLGTLVTVSS

SEQ ID NO: 128 - protein, 118 aa, Artificial Sequence
  Synthetic Construct
VQLVESGGGVVRPGESLRLSCAASGFTFSSYDMNWVRQAPGEGLEWVSLISGSGEIIYYADSVKGRFTISRDNSKNTLYLQMNSLRAEDTAVYYCAKENNRYRFFDDWGLGTLVTVSS

SEQ ID NO: 129 - protein, 118 aa, Artificial Sequence
  Synthetic Construct
VQLVESGGGVVRPGESLRLSCAASGFTFSNYAMNWVRQAPGEGLEWVSGISGRGGDTYYADSVKGRFTISRDNSKNTLYLQMNSLRAEDTAIYYCAKGTWNYGSFDYWGLGTLVTVSS

SEQ ID NO: 130 - protein, 119 aa, Artificial Sequence
  Synthetic Construct
VQLVESGGGVVQPGGSLRLSCAASGFSFSNFAMTWVRQAPGEGLEWVSTIGSGDTYYADSVKGRFTISRDNSKNTLYLQMNSLRAEDTAVYYCAKDSTVSWSGDFFDYWGLGTLVTVSS

SEQ ID NO: 131 - protein, 102 aa, Homo sapiens
APVVSGPAARATPQHTVSFTCESHGFSPRDITLKWFKNGNELSDFQTNVDPVGESVSYSIHSTAKVVLTREDVHSQVICEVAHVTLQGDPLRGTANLSETIR

SEQ ID NO: 132 - protein, 99 aa, Homo sapiens
VPPTLEVTQQPVRAENQVNVTCQVRKFYPQRLQLTWLENGNVSRTETASTVTENKDGTYNWMSWLLVNVSAHRDDVKLTCQVEHDGQPAVSKSHDLKVS

SEQ ID NO: 133 - protein, 119 aa, Artificial Sequence
  Synthetic Construct
DVQLVESGGGVVRPGESLRLSCAASGFTFSSYDMNWVRQAPGEGLEWVSLISGSGEIIYYADSVKGRFTISRDNSKNTLYLQMNSLRAEDTAVYYCAKENNRYRFFDDWGLGTLVTVSS

SEQ ID NO: 134 - protein, 108 aa, Artificial Sequence
  Synthetic Construct
ETVLTQSPGTLTLSPGERATLTCRASQSVYTYLAWYQEKPGQAPRLLIYGASSRATGIPDRFSGSGSGTEFTLTISSLQSEDFAVYYCQQYYDRPPLTFGGGTKVEIK

SEQ ID NO: 135 - protein, 118 aa, Artificial Sequence
  Synthetic Construct
DVQLVESGGGVVRPGESLRLSCAASGFTFSSNAMSWVRQAPGKGLEWLAGISAGGSDTYYPASVKGRFTISRDNSKNTLYLQMNTLTAEDTAVYYCARETWNHLFDYWGLGTLVTVSS

SEQ ID NO: 136 - protein, 107 aa, Artificial Sequence
  Synthetic Construct
ALTQPASVSANPGETVKIACSGGDYYSYYYGWYQQKAPGSALVTVIYSDDKRPSDIPSRFSGSASGSTATLTITGVRAEDEAVYYCGGYDYSTYANAFGAGTTLTVL

SEQ ID NO: 137 - protein, 117 aa, Artificial Sequence
  Synthetic Construct
DVQLVESGGGVVRPGESLRLSCEASGFTFSSNAMSWVRQAPGKGLEWVAGISSGSDTYYGDSVKGRLTISRDNSKNILYLQMNSLTAEDTAVYYCARETWNHLFDYWGLGTLVTVSS

SEQ ID NO: 138 - protein, 107 aa, Artificial Sequence
  Synthetic Construct
ALTQPASVSANPGETVEITCSGGSYSSYYYAWYQQKSPGSAPVTLIYSDDKRPSNIPSRFSGSASGSTATLTITGVRAEDEAVYFCGGYDQSSYTNPFGAGTTLTVL

SEQ ID NO: 139 - protein, 117 aa, Artificial Sequence
  Synthetic Construct
DVQLVESGGGVVRPGESLRLSCAVSGFRFSSYAMSWVRQAPGKGLEWVSGISSGGDTYYVDSVKGRFTISRDNSKNTLYLQVNSLTAEDTAIYYCARETWNHLFDYWGLGTLVTVSS

SEQ ID NO: 140 - protein, 107 aa, Artificial Sequence
  Synthetic Construct
ALTQPASVSADLGETVKITCSGGDSSSHYYGWYQQKSPGSAPVTVIYSDDERPSDIPSRFSGSASGSTATLTITGVRVEDEAIYYCGAYDGSTYANTFGAGTTLTVL

SEQ ID NO: 141 - protein, 118 aa, Artificial Sequence
  Synthetic Construct
DVQLVESGGGVVRPGESLRLSCAASGFTFSSYAMSWVRQAPGKGLEWLAGISAGGSDTYYIDSVKGRFTISRDNPKNSLYLQMSSLTAEDTAVYYCARETWNHLFDYWGLGTLVTVSS

SEQ ID NO: 142 - protein, 107 aa, Artificial Sequence
  Synthetic Construct
ALTQPASVSANPGETVKITCSGGDYYSTYYAWYQQKSPGSAPVTVIHSDDKRPSDIPSRFSGSASGSAATLIITGVRVEDEAVYYCGGYDGRTYINTFGAGTTLTVL

SEQ ID NO: 143 - protein, 10 aa, Artificial Sequence
  Synthetic Construct
GFSFSNFAMT

SEQ ID NO: 144 - protein, 15 aa, Artificial Sequence
  Synthetic Construct
TIGSGDTYYADSVKG

SEQ ID NO: 145 - protein, 13 aa, Artificial Sequence
  Synthetic Construct
DSTVSWSGDFFDY

SEQ ID NO: 146 - protein, 11 aa, Artificial Sequence
  Synthetic Construct
RASQNVKNDLA

SEQ ID NO: 147 - protein, 7 aa, Artificial Sequence
  Synthetic Construct
AARIRET

SEQ ID NO: 148 - protein, 10 aa, Artificial Sequence
  Synthetic Construct
QQYYDWPPFT

SEQ ID NO: 149 - protein, 10 aa, Artificial Sequence
  Synthetic Construct
GFSFSIYAMS

SEQ ID NO: 150 - protein, 15 aa, Artificial Sequence
  Synthetic Construct
TIGADDTYYADSVKG

SEQ ID NO: 151 - protein, 13 aa, Artificial Sequence
  Synthetic Construct
DSTVGWSGDFFDY

SEQ ID NO: 152 - protein, 11 aa, Artificial Sequence
  Synthetic Construct
RASQNVRSDIA

SEQ ID NO: 153 - protein, 7 aa, Artificial Sequence
  Synthetic Construct
AASSRDT

SEQ ID NO: 154 - skipped

SEQ ID NO: 155 - protein, 10 aa, Artificial Sequence
  Synthetic Construct
GFTFSSYDMN

SEQ ID NO: 156 - protein, 17 aa, Artificial Sequence
  Synthetic Construct
LISGSGEIIYYADSVKG

SEQ ID NO: 157 - protein, 10 aa, Artificial Sequence
  Synthetic Construct
ENNRYRFFDD

SEQ ID NO: 158 - protein, 11 aa, Artificial Sequence
  Synthetic Construct
RASQSVYTYLA

SEQ ID NO: 159 - protein, 7 aa, Artificial Sequence
  Synthetic Construct
GASSRAT

SEQ ID NO: 160 - protein, 10 aa, Artificial Sequence
  Synthetic Construct
QQYYDRPPLT

SEQ ID NO: 161 - protein, 8 aa, Artificial Sequence
  Synthetic Construct
GFTFSSNA

SEQ ID NO: 162 - protein, 8 aa, Artificial Sequence
  Synthetic Construct
ISAGGSDT

SEQ ID NO: 163 - protein, 11 aa, Artificial Sequence
  Synthetic Construct
ARETWNHLFDY

SEQ ID NO: 164 - protein, 11 aa, Artificial Sequence
  Synthetic Construct
SGGDYYSYYYG

SEQ ID NO: 165 - protein, 12 aa, Artificial Sequence
  Synthetic Construct
TVIYSDDKRPSD

SEQ ID NO: 166 - protein, 11 aa, Artificial Sequence
  Synthetic Construct
GGYDYSTYANA

SEQ ID NO: 167 - skipped

SEQ ID NO: 168 - protein, 7 aa, Artificial Sequence
  Synthetic Construct
ISSGSDT

SEQ ID NO: 169 - skipped

SEQ ID NO: 170 - protein, 11 aa, Artificial Sequence
  Synthetic Construct
SGGSYSSYYYA

SEQ ID NO: 171 - protein, 12 aa, Artificial Sequence
  Synthetic Construct
TLIYSDDKRPSN

SEQ ID NO: 172 - protein, 11 aa, Artificial Sequence
  Synthetic Construct
GGYDQSSYTNP

SEQ ID NO: 173 - protein, 8 aa, Artificial Sequence
  Synthetic Construct
GFRFSSYA

SEQ ID NO: 174 - protein, 7 aa, Artificial Sequence
  Synthetic Construct
ISSGGDT

SEQ ID NO: 175 - protein, 5 aa, Artificial Sequence
  Synthetic Construct
NFAMT

SEQ ID NO: 176 - protein, 11 aa, Artificial Sequence
  Synthetic Construct
SGGDSSSHYYG

SEQ ID NO: 177 - protein, 12 aa, Artificial Sequence
  Synthetic Construct
TVIYSDDERPSD

SEQ ID NO: 178 - protein, 11 aa, Artificial Sequence
  Synthetic Construct
GAYDGSTYANT

SEQ ID NO: 179 - protein, 8 aa, Artificial Sequence
  Synthetic Construct
GFTFSSYA

SEQ ID NO: 180-181 - skipped (2 entries)

SEQ ID NO: 182 - protein, 11 aa, Artificial Sequence
  Synthetic Construct
SGGDYYSTYYA

SEQ ID NO: 183 - protein, 12 aa, Artificial Sequence
  Synthetic Construct
TVIHSDDKRPSD

SEQ ID NO: 184 - protein, 11 aa, Artificial Sequence
  Synthetic Construct
GGYDGRTYINT

SEQ ID NO: 185 - protein, 10 aa, Artificial Sequence
  Synthetic Construct
  VARIANT 6: Xaa = Asn or Ile
  VARIANT 7: Xaa = Phe or Tyr
  VARIANT 10: Xaa = Thr or Ser
GFSFSXXAMX

SEQ ID NO: 186 - protein, 15 aa, Artificial Sequence
  Synthetic Construct
  VARIANT 4: Xaa = Ser or Ala
  VARIANT 5: Xaa = Gly or Asp
TIGXXDTYYADSVKG

SEQ ID NO: 187 - protein, 13 aa, Artificial Sequence
  Synthetic Construct
  VARIANT 5: Xaa = Ser or Gly
DSTVXWSGDFFDY

SEQ ID NO: 188 - protein, 11 aa, Artificial Sequence
  Synthetic Construct
  VARIANT 7: Xaa = Lys or Arg
  VARIANT 8: Xaa = Asn or Ser
  VARIANT 10: Xaa = Leu or Ile
RASQNVXXDXA

SEQ ID NO: 189 - protein, 7 aa, Artificial Sequence
  Synthetic Construct
  VARIANT 3: Xaa = Arg or Ser
  VARIANT 4: Xaa = Ile or Ser
  VARIANT 6: Xaa = Glu or Asp
AAXXRXT

SEQ ID NO: 190 - protein, 9 aa, Artificial Sequence
  Synthetic Construct
GGYDYSTYA

SEQ ID NO: 191 - protein, 7 aa, Artificial Sequence
  Synthetic Construct
GFTFSSN

SEQ ID NO: 192 - protein, 6 aa, Artificial Sequence
  Synthetic Construct
SAGGSD

SEQ ID NO: 193 - protein, 9 aa, Artificial Sequence
  Synthetic Construct
ETWNHLFDY

SEQ ID NO: 194 - protein, 5 aa, Artificial Sequence
  Synthetic Construct
SNAMS

SEQ ID NO: 195 - protein, 17 aa, Artificial Sequence
  Synthetic Construct
GISAGGSDTYYPASVKG

SEQ ID NO: 196 - protein, 5 aa, Artificial Sequence
  Synthetic Construct
SSGSD

SEQ ID NO: 197 - protein, 16 aa, Artificial Sequence
  Synthetic Construct
GISSGSDTYYGDSVKG

SEQ ID NO: 198 - protein, 7 aa, Artificial Sequence
  Synthetic Construct
GFRFSSY

SEQ ID NO: 199 - protein, 5 aa, Artificial Sequence
  Synthetic Construct
SSGGD

SEQ ID NO: 200 - protein, 5 aa, Artificial Sequence
  Synthetic Construct
SYAMS

SEQ ID NO: 201 - protein, 16 aa, Artificial Sequence
  Synthetic Construct
GISSGGDTYYVDSVKG

SEQ ID NO: 202 - protein, 7 aa, Artificial Sequence
  Synthetic Construct
GFSFSNF

SEQ ID NO: 203 - protein, 4 aa, Artificial Sequence
  Synthetic Construct
GSGD

SEQ ID NO: 204 - protein, 5 aa, Artificial Sequence
  Synthetic Construct
NFAVT

SEQ ID NO: 205 - protein, 8 aa, Artificial Sequence
  Synthetic Construct
GFSFSNFA

SEQ ID NO: 206 - protein, 6 aa, Artificial Sequence
  Synthetic Construct
IGSGDT

SEQ ID NO: 207 - protein, 15 aa, Artificial Sequence
  Synthetic Construct
AKDSTVSWSGDFFDY

SEQ ID NO: 208 - protein, 6 aa, Artificial Sequence
  Synthetic Construct
QNVKND

SEQ ID NO: 209 - protein, 3 aa, Artificial Sequence
  Synthetic Construct
AAR

SEQ ID NO: 210 - protein, 7 aa, Artificial Sequence
  Synthetic Construct
QQYYDWP

SEQ ID NO: 211 - protein, 7 aa, Artificial Sequence
  Synthetic Construct
GFSFSIY

SEQ ID NO: 212 - protein, 4 aa, Artificial Sequence
  Synthetic Construct
GADD

SEQ ID NO: 213 - protein, 5 aa, Artificial Sequence
  Synthetic Construct
IYAVS

SEQ ID NO: 214 - protein, 8 aa, Artificial Sequence
  Synthetic Construct
GFSFSIYA

SEQ ID NO: 215 - protein, 6 aa, Artificial Sequence
  Synthetic Construct
IGADDT

SEQ ID NO: 216 - protein, 15 aa, Artificial Sequence
  Synthetic Construct
AKDSTVGWSGDFFDY

SEQ ID NO: 217 - protein, 6 aa, Artificial Sequence
  Synthetic Construct
QNVRSD

SEQ ID NO: 218 - protein, 3 aa, Artificial Sequence
  Synthetic Construct
AAS

SEQ ID NO: 219 - protein, 7 aa, Artificial Sequence
  Synthetic Construct
GFTFSSY

SEQ ID NO: 220 - protein, 6 aa, Artificial Sequence
  Synthetic Construct
SGSGEI

SEQ ID NO: 221 - protein, 5 aa, Artificial Sequence
  Synthetic Construct
SYDVN

SEQ ID NO: 222 - protein, 8 aa, Artificial Sequence
  Synthetic Construct
GFTFSSYD

SEQ ID NO: 223 - protein, 8 aa, Artificial Sequence
  Synthetic Construct
ISGSGEII

SEQ ID NO: 224 - protein, 12 aa, Artificial Sequence
  Synthetic Construct
AKENNRYRFFDD

SEQ ID NO: 225 - protein, 6 aa, Artificial Sequence
  Synthetic Construct
QSVYTY

SEQ ID NO: 226 - protein, 3 aa, Artificial Sequence
  Synthetic Construct
GAS

SEQ ID NO: 227 - protein, 5 aa, Artificial Sequence
  Synthetic Construct
DYGMN

SEQ ID NO: 228 - protein, 16 aa, Artificial Sequence
  Synthetic Construct
QITSGSRTYYGAAVKG

SEQ ID NO: 229 - protein, 11 aa, Artificial Sequence
  Synthetic Construct
DFGSGVGSIDA

SEQ ID NO: 230 - protein, 7 aa, Artificial Sequence
  Synthetic Construct
GFIFSDY

SEQ ID NO: 231 - protein, 5 aa, Artificial Sequence
  Synthetic Construct
TSGSR

SEQ ID NO: 232 - protein, 8 aa, Artificial Sequence
  Synthetic Construct
SGSRGRYG

SEQ ID NO: 233 - protein, 7 aa, Artificial Sequence
  Synthetic Construct
RDNQRPS

SEQ ID NO: 234 - protein, 9 aa, Artificial Sequence
  Synthetic Construct
GSYDGSIDI

SEQ ID NO: 235 - protein, 5 aa, Artificial Sequence
  Synthetic Construct
SYAMG

SEQ ID NO: 236 - protein, 17 aa, Artificial Sequence
  Synthetic Construct
GIDDDGSTANYGPAVKG

SEQ ID NO: 237 - protein, 16 aa, Artificial Sequence
  Synthetic Construct
ASVTGWSAHISGRLDT

SEQ ID NO: 238 - protein, 5 aa, Artificial Sequence
  Synthetic Construct
DDGST

SEQ ID NO: 239 - protein, 9 aa, Artificial Sequence
  Synthetic Construct
SGGGIYYYG

SEQ ID NO: 240 - protein, 7 aa, Artificial Sequence
  Synthetic Construct
ENDKRPS

SEQ ID NO: 241 - protein, 11 aa, Artificial Sequence
  Synthetic Construct
GGYDSNTTSGI

SEQ ID NO: 242 - protein, 119 aa, Artificial Sequence
  Synthetic Construct
AVTLDESGGGLQTPGGALSLVCKASGFIFSDYGMNWVRQAPGKGLEFVAQITSGSRTYYGAAVKGRATISRDNRQSTVKLQLNNLRAEDTGIYFCARDFGSGVGSIDAWGNGTEVIVSS

SEQ ID NO: 243 - protein, 102 aa, Artificial Sequence
  Synthetic Construct
ALTQPASVSANLGGTVKITCSGSRGRYGWYQQRSPGSAPVTVIYRDNQRPSNIPSRFSSSTSGSTSTLTITGVQADDESVYFCGSYDGSIDIFGAGTTLTVL

SEQ ID NO: 244 - protein, 125 aa, Artificial Sequence
  Synthetic Construct
AVTLDESGGGLQTPGGALSLVCKASGFTFSSYAMGWVRQAPGKGLEWVAGIDDDGSTANYGPAVKGRATISRDNGQSTVRLQLNNPRAEDSGTYFCAKASVTGWSAHISGRLDTWGHGTEVIVSS

SEQ ID NO: 245 - protein, 105 aa, Artificial Sequence
  Synthetic Construct
ALTQPASVSANPGETVKITCSGGGIYYYGWYQQKSPGSAPVTLIYENDKRPSDIPSRFSGSTSGSTNTFTITGVQAEDEAVYYCGGYDSNTTSGIFGAGTTLTVL

SEQ ID NO: 246 - protein, 120 aa, Artificial Sequence
  Synthetic Construct
EVQLLESGGGVVQPGGSLRLSCAASGFSFSNFAVTWVRQAPGKGLEWVSTIGSGDTYYADSVKGRFTISRDNSKNTLYLQMNSLRAEDTAVYYCAKDSTVSWSGDFFDYWGQGTLVTVSS

SEQ ID NO: 247 - protein, 120 aa, Artificial Sequence
  Synthetic Construct
EVQLVESGGGVVQPGGSLRLSCAASGFSFSIYAVSWVRQAPGKGLEWVSTIGADDTYYADSVKGRFTISRDNSKNTLYLQMNSLRAEDTAVYYCAKDSTVGWSGDFFDYWGQGTLVTVSS

SEQ ID NO: 248 - protein, 108 aa, Artificial Sequence
  Synthetic Construct
EIVLTQSPATLSVSPGERVTLSCRASQNVRSDIAWYQQKPGQAPRLLIYAASSRDTGIPARFSGSGSGTDFTLTISSLQSEDFGVYYCQQYYDWPPFTFGGGTKVEIK

SEQ ID NO: 249 - protein, 119 aa, Artificial Sequence
  Synthetic Construct
EVQLVESGGGVVQPGRSLRLSCAASGFTFSSYDVNWVRQAPGKGLEWVSLISGSGEIIYYADSVKGRFTISRDNSKNTLYLQMNSLRAEDTAVYYCAKENNRYRFFDDWGQGTLVTVSS

SEQ ID NO: 250 - protein, 108 aa, Artificial Sequence
  Synthetic Construct
EIVLTQSPGTLSLSPGERATLSCRASQSVYTYLAWYQQKPGQAPRLLIYGASSRATGIPDRFSGSGSGTEFTLTISSLQSEDFAVYYCQQYYDRPPLTFGGGTKVEIK

SEQ ID NO: 251 - protein, 108 aa, Artificial Sequence
  Synthetic Construct
ETVLTQSPGTLSLSPGERATLSCRASQSVYTYLAWYQQKPGQAPRLLIYGASSRATGIPDRFSGSGSGTEFTLTISSLQSEDFAVYYCQQYYDRPPLTFGGGTKVEIK

SEQ ID NO: 252 - protein, 108 aa, Artificial Sequence
  Synthetic Construct
SYELTQPPSVSVSPGQTARITCSGGSYSSYYYAWYQQKPGQAPVTLIYSDDKRPSNIPERFSGSSSGTTVTLTISGVQAEDEADYYCGGYDQSSYTNPFGGGTKLTVL

SEQ ID NO: 253 - protein, 108 aa, Artificial Sequence
  Synthetic Construct
QSVLTQPPSVSAAPGQKVTISCSGGSYSSYYYAWYQQLPGTAPKTLIYSDDKRPSNIPDRFSGSKSGTSATLGITGLQTGDEADYYCGGYDQSSYTNPFGTGTKVTVL

SEQ ID NO: 254 - protein, 108 aa, Artificial Sequence
  Synthetic Construct
SYELTQPPSVSVSPGQTARITCSGGDYYSTYYAWYQQKPGQAPVTVIHSDDKRPSDIPERFSGSSSGTTVTLTISGVQAEDEADYYCGGYDGRTYINTFGGGTKLTVL

SEQ ID NO: 255 - protein, 108 aa, Artificial Sequence
  Synthetic Construct
QSVLTQPPSVSAAPGQKVTISCSGGDYYSTYYAWYQQLPGTAPKTVIHSDDKRPSDIPDRFSGSKSGTSATLGITGLQTGDEADYYCGGYDGRTYINTFGTGTKVTVL

SEQ ID NO: 256 - protein, 113 aa, Artificial Sequence
  Synthetic Construct
QSALTQPASVSGSPGQSITISCTGTSSDVGSYSSYYYAWYQQHPGKAPKTLIYSDDKRPSNVSNRFSGSKSGNTASLTISGLQAEDEADYYCGGYDQSSYTNPFGGGTKLTVL

SEQ ID NO: 257 - protein, 108 aa, Artificial Sequence
  Synthetic Construct
QSVLTQPPSVSAAPGQKVTISCSGGDYYSYYYGWYQQLPGTAPKTVIYSDDKRPSDIPDRFSGSKSGTSATLGITGLQTGDEADYYCGGYDYSTYANAFGTGTKVTVL

SEQ ID NO: 258 - protein, 120 aa, Artificial Sequence
  Synthetic Construct
EVQLLESGGGVVQPGGSLRLSCAASGFSFSNFAMTWVRQAPGKGLEWVSTIGSGDTYYADSVKGRFTISRDNSKNTLYLQMNSLRAEDTAVYYCAKDSTVSWSGDFFDYWGQGTLVTVSS

SEQ ID NO: 259 - protein, 120 aa, Artificial Sequence
  Synthetic Construct
EVQLVESGGGVVQPGGSLRLSCAASGFSFSIYAMSWVRQAPGKGLEWVSTIGADDTYYADSVKGRFTISRDNSKNTLYLQMNSLRAEDTAVYYCAKDSTVGWSGDFFDYWGQGTLVTVSS

SEQ ID NO: 260 - protein, 119 aa, Artificial Sequence
  Synthetic Construct
EVQLVESGGGVVQPGRSLRLSCAASGFTFSSYDMNWVRQAPGKGLEWVSLISGSGEIIYYADSVKGRFTISRDNSKNTLYLQMNSLRAEDTAVYYCAKENNRYRFFDDWGQGTLVTVSS

SEQ ID NO: 261 - protein, 11 aa, Artificial Sequence
  Synthetic Construct
SGGAYSSYYYA

SEQ ID NO: 262 - protein, 108 aa, Artificial Sequence
  Synthetic Construct
SYELTQPPSVSVSPGQTARITCSGGAYSSYYYAWYQQKPGQAPVLVIYSDDKRPSGIPERFSGSSSGTTVTLTISGVQAEDEADYYCGGYDQSSYTNPFGGGTKLTVL

SEQ ID NO: 263 - protein, 118 aa, Artificial Sequence
  Synthetic Construct
EVQLVESGGGVVQPGGSLRLSCAASGFTFSSNAMSWVRQAPGKGLEWVAGISAGGSDTYYPASVKGRFTISRDNSKNTLYLQMNSLRAEDTAVYYCARETWNHLFDYWGQGTLVTVSS

SEQ ID NO: 264 - protein, 118 aa, Artificial Sequence
  Synthetic Construct
EVQLVESGGGVVQPGGSLRLSCAASGFTFSSNAVSWVRQAPGKGLEWVAGISAGGSDTYYPASVKGRFTISRDNSKNTLYLQMNSLRAEDTAVYYCARETWNHLFDYWGQGTLVTVSS

SEQ ID NO: 265 - protein, 117 aa, Artificial Sequence
  Synthetic Construct
EVQLVESGGGVVQPGGSLRLSCAASGFTFSSNAMSWVRQAPGKGLEWVAGISSGSDTYYGDSVKGRFTISRDNSKNTLYLQMNSLTAEDTAVYYCARETWNHLFDYWGQGTLVTVSS

SEQ ID NO: 266 - protein, 117 aa, Artificial Sequence
  Synthetic Construct
EVQLVESGGGVVQPGGSLRLSCAASGFTFSSNAVSWVRQAPGKGLEWVAGISSGSDTYYGDSVKGRFTISRDNSKNTLYLQMNSLTAEDTAVYYCARETWNHLFDYWGQGTLVTVSS

SEQ ID NO: 267 - protein, 117 aa, Artificial Sequence
  Synthetic Construct
EVQLVESGGGVVQPGGSLRLSCAASGFRFSSYAMSWVRQAPGKGLEWVSGISSGGDTYYVDSVKGRFTISRDNSKNTLYLQMNSLRAEDTAVYYCARETWNHLFDYWGQGTLVTVSS

SEQ ID NO: 268 - protein, 117 aa, Artificial Sequence
  Synthetic Construct
EVQLVESGGGVVQPGGSLRLSCAASGFRFSSYAVSWVRQAPGKGLEWVSGISSGGDTYYVDSVKGRFTISRDNSKNTLYLQMNSLRAEDTAVYYCARETWNHLFDYWGQGTLVTVSS

SEQ ID NO: 269 - protein, 5 aa, Artificial Sequence
  Synthetic Construct
IYAMS

SEQ ID NO: 270 - protein, 5 aa, Artificial Sequence
  Synthetic Construct
SYDMN

SEQ ID NO: 271 - protein, 5 aa, Artificial Sequence
  Synthetic Construct
SNAVS

SEQ ID NO: 272 - protein, 5 aa, Artificial Sequence
  Synthetic Construct
SYAVS

SEQ ID NO: 273 - protein, 119 aa, Artificial Sequence
  Synthetic Construct
DVQLVESGGGVVRPGESLRLSCAASGFSFSSYAMNWVRQAPGEGLEWVSRINSGGGGTDYAESVKGRFTISRDNSENTLYLQMNSLRAEDTAVYYCAKQYDWNSFFDYWGLGALVTVSS

SEQ ID NO: 274 - protein, 108 aa, Artificial Sequence; identical to SEQ ID NO: 93
  Synthetic Construct

SEQ ID NO: 275 - protein, 119 aa, Artificial Sequence
  Synthetic Construct
DVQLVESGGGVVRPGESLRLSCEASGFTFRNYYMTWVRQAPGEGLEWVSTISDTGDTAYYADSVKGRFTISRDNSKNSLYLQMNSLRADDTAIYYCAKSWIWWTFFDYWGLGTLVTVSS

SEQ ID NO: 276 - protein, 103 aa, Artificial Sequence
  Synthetic Construct
ALTQPASVSANLGGTVEITCSGGNSNHYGWYQQKSPGSAPVTLIYADTNRPSNIPSRFSGSTSGSTTTLTITGVQAEDEAVYYCGGSSTGDGIFGAGTTLTVL

SEQ ID NO: 277 - skipped

SEQ ID NO: 278 - protein, 118 aa, Artificial Sequence
  Synthetic Construct
DVQLVESGGGVVRPGESLRLSCAASGFAFSDHDMSWVRQGPGEGLEWVAGISLRGGVTWYADSVKGRFTISRDNSKNTLYLRLFSLRTEDTAIYYCARESWNTFFDYWGLGTLVTVSS

SEQ ID NO: 279 - protein, 108 aa, Artificial Sequence
  Synthetic Construct
EIVLTQSPGTLSLSPGETATLSCRASQNVRSNLAWYQQKPGQAPRLLIYDASSRATGIPDRFSGSGSGTDFTLTISSLQSEDFAVYYCQQYGNGPPLTFGGGTKVEIK

SEQ ID NO: 280 - protein, 121 aa, Artificial Sequence
  Synthetic Construct
DVQLVESGGAVVRPGESLRLSCKASGFTFTNFAMSWVRQAPGEGLEWVSGISGSDDTTYYADSVKGRFTISRDNSESTLYLQMNSLRAEDTAVYYCVKDSTVSWNTFFDYWGLGTLVTVSS

SEQ ID NO: 281 - protein, 110 aa, Artificial Sequence
  Synthetic Construct
ALTQPASVSANLGGTVKITCSGGYGSDDGSSSYYGWYQQKSPGSAPVILIYWDDKRPSDIPSRFSGSTSGSTTTLTITGVQAEDEAVYFCGTYDTSSGAIFGAGTTLTVL

SEQ ID NO: 282 - protein, 119 aa, Artificial Sequence
  Synthetic Construct
DVQLVESGGGVVRPGESLRLSCAASGFSFRSYAMNWVRQAPGEGLEWVSRINSGGGGTDYADSVKGRFTISRDNSKNTLYLQMNSLRAEDTAVYYCAKQYDWNSFFDYWGLGALVTVSS

SEQ ID NO: 283 - protein, 108 aa, Artificial Sequence
  Synthetic Construct
ETVLTQSPATLSVSPGERATLSCRASQTVGSKLAWHQQKPGQAPRLLIYDASNRATGIPDRFSGSGSGTDFTLTISSPQTEDSAVYYCQQYYYWPPYRFGGGTKVEIK

SEQ ID NO: 284 - protein, 114 aa, Artificial Sequence
  Synthetic Construct
DVQLVESGGGVVRPGESLTLSCTASGFTFTSSTMNWVRQAPGEGLDWVSSISTSGVITYYADSVKGRATISRDNSKNTLYLRLFSLRADDTAIYYCATDTFDHWGPGTLVTVSS

SEQ ID NO: 285 - protein, 102 aa, Artificial Sequence
  Synthetic Construct
ALTQPASVSANPGETVKITCFGSSGNYGWFQQKSPGSAPVTVIHYNNKRPSDIPSRFSGSKSGSTGTLTITGVRAEDEAVYFCGAWETGSATFGAGTTLTVL

SEQ ID NO: 286 - protein, 117 aa, Artificial Sequence
  Synthetic Construct
DVQLVESGGGVVRPGESLRLSCAASGFTFSNFAMNWVRQAPGEGLEWVSLISVTATTYYADSVKGRFTISRDNSKNTLYLQMNSLRAEDTAVYYCAKVTWNNLFDYWGLGTLVTVSS

SEQ ID NO: 287 - protein, 108 aa, Artificial Sequence
  Synthetic Construct
EIVLTQSPGTLSLSPGERATLSCRASQPIDSYLAWYQQKPGQAPRLLIYNTVTRATGIPDRFSGSGSGTDFTLTINRLEPEDFAVYYCQHQYDWPPYIFGGGTKVEIK

SEQ ID NO: 288 - protein, 117 aa, Artificial Sequence
  Synthetic Construct
DVQLVESGGGVVRPGESLRLSCAASGFTFSNFAMTWVRQAPGKGPEWVSLVSVTATTYYADSVKGRFTISRDNSKSTLYLQMNSLRAEDTAVYYCAKITWNNLFDYWGLGTLVTVSS

SEQ ID NO: 289 - protein, 108 aa, Artificial Sequence
  Synthetic Construct
EIVLTQSPGTLSLSPGERATLSCRASQTVGSKLAWYQQKPGQAPRLLIYDSSSRASGIPDRFSGSGSGTDFTLTISSLQSEDSAVYYCQQHNDWPPYTFGGGTKVEIK

SEQ ID NO: 290 - protein, 117 aa, Artificial Sequence
  Synthetic Construct
DVQLVESGGGLVRPGESLRLSCAASGFTFTNYAVTWVRQAPGEGLEWVSLISVTGTTYYADSVKGRFTISRDNSKSTLYLQMNSLRAEDTAVYYCAKVTWKNVFDYWGLGTLVTVSS

SEQ ID NO: 291 - protein, 108 aa, Artificial Sequence
  Synthetic Construct
EIVLTQSPGTLSVSPGERATFSCRASQTVGSKLAWYQQKPGQAPRLLIYDANTRATGIPARFSGSGSGTEFTLTISSLQSEDFAVYYCQQHTDWPPYTFGGGTKVEIK

SEQ ID NO: 292 - protein, 117 aa, Artificial Sequence
  Synthetic Construct
DVQLVESGGGVVRPGESLRLSCAASGFTFRNYGMSWVRQAPGEGLEWVSASSGSGSTYYADSVKGRFTISRDNSKNTLYLQMNSLRAEDTAIYYCAKVTWNNFFDYWGLGTLVTVSS

SEQ ID NO: 293 - protein, 108 aa, Artificial Sequence
  Synthetic Construct
EIVLAQSPDTLSVSPGERATLTCRASQDVAGKLAWYQQKPGQAPRLLIHATSSRADGIPARFSGSGSGTEFTLTITGLQSEDFAVYYCQQHYDWSPLTFGGGTKVEIK

SEQ ID NO: 294 - protein, 117 aa, Artificial Sequence; identical to SEQ ID NO: 139
  Synthetic Construct

SEQ ID NO: 295 - protein, 107 aa, Artificial Sequence
  Synthetic Construct
ALTQPASVSANLGETVKITCSGGDSSSHYYGWYQQKSPGSAPVTVIYSDDERPSDIPSRFSGSASGSTATLTITGVRVEDEAIYYCGAYDGSTYANTFGAGTTLTVL

SEQ ID NO: 296 - protein, 127 aa, Artificial Sequence
  Synthetic Construct
EEELQVIQPDKSVLVAAGETATLRCTATSLIPVGPIQWFRGAGPGRELIYNQKEGHFPRVTTVSDLTKRNNMDFSIRIGAITPADAGTYYCVKFRKGSPDDVEFKSGAGTELSVRAKPSTRHHHHHH

SEQ ID NO: 297 - protein, 5 aa, Artificial Sequence
  Synthetic Construct
  VARIANT 1: Xaa = Ser or Thr
  VARIANT 2: Xaa = Asn or Tyr or His or Asp
  VARIANT 4: Xaa = Met or Leu or Val
XXAXS

SEQ ID NO: 298 - protein, 17 aa, Artificial Sequence
  Synthetic Construct
  VARIANT 4: Xaa = Ala or Ser
  VARIANT 5: Xaa = Gly or Ser or absent
  VARIANT 6: Xaa = Ser or Asp or Gly
  VARIANT 7: Xaa = Gly or Ser
  VARIANT 8: Xaa = Asp or Ser or Gly
  VARIANT 9: Xaa = Thr or Ala
  VARIANT 12: Xaa = Pro or Gly or Val or Ile or Ala or Ser
  VARIANT 13: Xaa = Ala or Asp or Gly
  VARIANT 15: Xaa = Val or Met
GISXXXXXXYYXXSXKG

SEQ ID NO: 299 - protein, 11 aa, Artificial Sequence
  Synthetic Construct
  VARIANT 4: Xaa = Asp or Gly or Ser or Ile or absent
  VARIANT 5: Xaa = Ser or Trp or Gly or Tyr or Asp
  VARIANT 6: Xaa = Ser or Tyr or Thr or Asp
  VARIANT 8: Xaa = His or Thr or Ser or Tyr
  VARIANT 11: Xaa = Gly or Ala
SGGXXXSXYYX

SEQ ID NO: 300 - protein, 7 aa, Artificial Sequence
  Synthetic Construct
  VARIANT 3: Xaa = Asp or Asn
  VARIANT 4: Xaa = Glu or Lys or Gln
  VARIANT 7: Xaa = Ser or Pro
SDXXRPX

SEQ ID NO: 301 - protein, 11 aa, Artificial Sequence
  Synthetic Construct
  VARIANT 1: Xaa = Gly or Ala
  VARIANT 2: Xaa = Gly or Ala
  VARIANT 5: Xaa = Gly or Tyr or Gln or Ser or Ala
  VARIANT 6: Xaa = Ser or Arg or Thr
  VARIANT 7: Xaa = Thr or Ser
  VARIANT 9: Xaa = Ala or Ile or Val or Leu or Thr
  VARIANT 11: Xaa = Thr or Ala or Asp or Pro
XXYDXXXYXNX

SEQ ID NO: 302 - protein, 5 aa, Artificial Sequence
  Synthetic Construct
  VARIANT 2: Xaa = Asn or Tyr
  VARIANT 4: Xaa = Met or Leu or Val
SXAXS

SEQ ID NO: 303 - protein, 17 aa, Artificial Sequence
  Synthetic Construct
  VARIANT 4: Xaa = Ala or Ser
  VARIANT 6: Xaa = Gly or absent
  VARIANT 7: Xaa = Ser or Gly
  VARIANT 12: Xaa = Pro or Gly or Val
  VARIANT 13: Xaa = Ala or Asp
GISXGXXDTYYXXSVKG

SEQ ID NO: 304 - protein, 11 aa, Artificial Sequence
  Synthetic Construct
  VARIANT 4: Xaa = Ser or Ala
SGGXYSSYYYA

SEQ ID NO: 305 - protein, 5 aa, Artificial Sequence
  Synthetic Construct
NFALT

SEQ ID NO: 306 - protein, 5 aa, Artificial Sequence
  Synthetic Construct
IYALS

SEQ ID NO: 307 - protein, 5 aa, Artificial Sequence
  Synthetic Construct
  VARIANT 1: Xaa = Ser or Thr
  VARIANT 2: Xaa = Tyr or Ser
  VARIANT 4: Xaa = Met or Leu or Val
XXDXN

SEQ ID NO: 308 - protein, 17 aa, Artificial Sequence
  Synthetic Construct
  VARIANT 9: Xaa = Ile or Thr
LISGSGEIXYYADSVKG

SEQ ID NO: 309 - protein, 10 aa, Artificial Sequence
  Synthetic Construct
  VARIANT 2: Xaa = Asn or Asp
  VARIANT 3: Xaa = Asn or Asp
  VARIANT 4: Xaa = Arg or Met
  VARIANT 10: Xaa = Asp or Tyr
EXXXYRFFDX

SEQ ID NO: 310 - protein, 11 aa, Artificial Sequence
  Synthetic Construct
  VARIANT 3: Xaa = Ser or Asp
  VARIANT 8: Xaa = Thr or Ser
RAXQSVYXYLA

SEQ ID NO: 311 - protein, 7 aa, Artificial Sequence
  Synthetic Construct
  VARIANT 1: Xaa = Gly or Ala or Asp
  VARIANT 3: Xaa = Ser or Arg
  VARIANT 4: Xaa = Ser or Asn or Thr
  VARIANT 7: Xaa = Thr or Ala
XAXXRAX

SEQ ID NO: 312 - protein, 108 aa, Artificial Sequence
  Synthetic Construct
EIVLTQSPATLSVSPGERATLSCRASQNVKNDLAWYQQKPGQAPRLLIYAARIRETGIPARFSGSGSGTEFTLTISSLQSEDFAVYYCQQYYDWPPFTFGGGTKVEIK

SEQ ID NO: 313 - protein, 5 aa, Artificial Sequence
  Synthetic Construct
SYDLN

SEQ ID NO: 314 - protein, 22 aa, Homo sapiens
SYELTQPPSVSVSPGQTARITC

SEQ ID NO: 315 - protein, 15 aa, Homo sapiens
WYQQKPGQAPVTLIY

SEQ ID NO: 316 - protein, 32 aa, Homo sapiens
NIPERFSGSSSGTTVTLTISGVQAEDEADYYC

SEQ ID NO: 317 - protein, 10 aa, Homo sapiens
FGGGTKLTVL

SEQ ID NO: 318 - protein, 5 aa, Artificial Sequence
  Synthetic Construct
SNALS

SEQ ID NO: 319 - protein, 5 aa, Artificial Sequence
  Synthetic Construct
SYALS

SEQ ID NO: 320 - protein, 330 aa, Homo sapiens
ASTKGPSVFPLAPSSKSTSGGTAALGCLVKDYFPEPVTVSWNSGALTSGVHTFPAVLQSSGLYSLSSVVTVPSSSLGTQTYICNVNHKPSNTKVDKKVEPKSCDKTHTCPPCPAPELLGGPSVFLFPPKPKDTLMISRTPEVTCVVVDVSHEDPEVKFNWYVDGVEVHNAKTKPREEQYNSTYRVVSVLTVLHQDWLNGKEYKCKVSNKALPAPIEKTISKAKGQPREPQVYTLPPSREEMTKNQVSLTCLVKGFYPSDIAVEWESNGQPENNYKTTPPVLDSDGSFFLYSKLTVDKSRWQQGNVFSCSVMHEALHNHYTQKSLSLSPGK

SEQ ID NO: 321 - protein, 330 aa, Artificial Sequence
  Synthetic Construct
ASTKGPSVFPLAPSSKSTSGGTAALGCLVKDYFPEPVTVSWNSGALTSGVHTFPAVLQSSGLYSLSSVVTVPSSSLGTQTYICNVNHKPSNTKVDKKVEPKSCDKTHTCPPCPAPEAAGAPSVFLFPPKPKDTLMISRTPEVTCVVVDVSHEDPEVKFNWYVDGVEVHNAKTKPREEQYASTYRVVSVLTVLHQDWLNGKEYKCKVSNKALPAPIEKTISKAKGQPREPQVYTLPPSREEMTKNQVSLTCLVKGFYPSDIAVEWESNGQPENNYKTTPPVLDSDGSFFLYSKLTVDKSRWQQGNVFSCSVMHEALHNHYTQKSLSLSPGK

SEQ ID NO: 322 - protein, 326 aa, Homo sapiens
ASTKGPSVFPLAPCSRSTSESTAALGCLVKDYFPEPVTVSWNSGALTSGVHTFPAVLQSSGLYSLSSVVTVPSSNFGTQTYTCNVDHKPSNTKVDKTVERKCCVECPPCPAPPVAGPSVFLFPPKPKDTLMISRTPEVTCVVVDVSHEDPEVQFNWYVDGVEVHNAKTKPREEQFNSTFRVVSVLTVVHQDWLNGKEYKCKVSNKGLPAPIEKTISKTKGQPREPQVYTLPPSREEMTKNQVSLTCLVKGFYPSDIAVEWESNGQPENNYKTTPPMLDSDGSFFLYSKLTVDKSRWQQGNVFSCSVMHEALHNHYTQKSLSLSPGK

SEQ ID NO: 323 - protein, 326 aa, Artificial Sequence
  Synthetic Construct
ASTKGPSVFPLAPCSRSTSESTAALGCLVKDYFPEPVTVSWNSGALTSGVHTFPAVLQSSGLYSLSSVVTVPSSNFGTQTYTCNVDHKPSNTKVDKTVERKCCVECPPCPAPPVAGPSVFLFPPKPKDTLMISRTPEVTCVVVDVSHEDPEVQFNWYVDGVEVHNAKTKPREEQFNSTFRVVSVLTVVHQDWLNGKEYKCKVSNKGLPSSIEKTISKTKGQPREPQVYTLPPSREEMTKNQVSLTCLVKGFYPSDIAVEWESNGQPENNYKTTPPMLDSDGSFFLYSKLTVDKSRWQQGNVFSCSVMHEALHNHYTQKSLSLSPGK

SEQ ID NO: 324 - protein, 327 aa, Artificial Sequence
  Synthetic Construct
ASTKGPSVFPLAPCSRSTSESTAALGCLVKDYFPEPVTVSWNSGALTSGVHTFPAVLQSSGLYSLSSVVTVPSSSLGTKTYTCNVDHKPSNTKVDKRVESKYGPPCPPCPAPEFLGGPSVFLFPPKPKDTLMISRTPEVTCVVVDVSQEDPEVQFNWYVDGVEVHNAKTKPREEQFNSTYRVVSVLTVLHQDWLNGKEYKCKVSNKGLPSSIEKTISKAKGQPREPQVYTLPPSQEEMTKNQVSLTCLVKGFYPSDIAVEWESNGQPENNYKTTPPVLDSDGSFFLYSRLTVDKSRWQEGNVFSCSVMHEALHNHYTQKSLSLSLGK

SEQ ID NO: 325 - protein, 107 aa, Homo sapiens [sequence omitted]

SEQ ID NO: 326 - protein, 106 aa, Homo sapiens
GQPKANPTVTLFPPSSEELQANKATLVCLISDFYPGAVTVAWKADGSPVKAGVETTKPSKQSNNKYAASSYLSLTPEQWKSHRSYSCQVTHEGSTVEKTVAPTECS

SEQ ID NO: 327 - protein, 120 aa, Artificial Sequence
  Synthetic Construct
EVQLLESGGGVVQPGGSLRLSCAASGFSFSNFALTWVRQAPGKGLEWVSTIGSGDTYYADSVKGRFTISRDNSKNTLYLQMNSLRAEDTAVYYCAKDSTVSWSGDFFDYWGQGTLVTVSS

SEQ ID NO: 328 - protein, 120 aa, Artificial Sequence
  Synthetic Construct
EVQLVESGGGVVQPGGSLRLSCAASGFSFSIYALSWVRQAPGKGLEWVSTIGADDTYYADSVKGRFTISRDNSKNTLYLQMNSLRAEDTAVYYCAKDSTVGWSGDFFDYWGQGTLVTVSS

SEQ ID NO: 329 - protein, 119 aa, Artificial Sequence
  Synthetic Construct
EVQLVESGGGVVQPGRSLRLSCAASGFTFSSYDLNWVRQAPGKGLEWVSLISGSGEIIYYADSVKGRFTISRDNSKNTLYLQMNSLRAEDTAVYYCAKENNRYRFFDDWGQGTLVTVSS

SEQ ID NO: 330 - protein, 118 aa, Artificial Sequence
  Synthetic Construct
EVQLVESGGGVVQPGGSLRLSCAASGFTFSSNALSWVRQAPGKGLEWVAGISAGGSDTYYPASVKGRFTISRDNSKNTLYLQMNSLRAEDTAVYYCARETWNHLFDYWGQGTLVTVSS

SEQ ID NO: 331 - protein, 117 aa, Artificial Sequence
  Synthetic Construct
EVQLVESGGGVVQPGGSLRLSCAASGFTFSSNALSWVRQAPGKGLEWVAGISSGSDTYYGDSVKGRFTISRDNSKNTLYLQMNSLTAEDTAVYYCARETWNHLFDYWGQGTLVTVSS

SEQ ID NO: 332 - protein, 117 aa, Artificial Sequence
  Synthetic Construct
EVQLVESGGGVVQPGGSLRLSCAASGFRFSSYALSWVRQAPGKGLEWVSGISSGGDTYYVDSVKGRFTISRDNSKNTLYLQMNSLRAEDTAVYYCARETWNHLFDYWGQGTLVTVSS

SEQ ID NO: 333 - protein, 106 aa, Artificial Sequence
  Synthetic Construct
QSALTQPASVSGSPGQSITISCFGSSGNYGLVSWYQQHPGKAPKLMIYYNNKRPSGVSNRFSGSKSGNTASLTISGLQAEDEADYYCGAWETGSATFGGGTKLTVL

SEQ ID NO: 334 - protein, 103 aa, Artificial Sequence
  Synthetic Construct
SYELTQPPSVSVSPGQTASITCFGSSGNYGWYQQKPGQSPVLVIYYNNKRPSGIPERFSGSNSGNTATLTISGTQAMDEADYYCGAWETGSATFGGGTKLTVL

SEQ ID NO: 335 - protein, 120 aa, Artificial Sequence
  Synthetic Construct
DVQLLESGGGVVQPGGSLRLSCAASGFSFSNFAMTWVRQAPGEGLEWVSTIGSGDTYYADSVKGRFTISRDNSKNTLYLQMNSLRAEDTAVYYCAKDSTVSWSGDFFDYWGLGTLVTVSS

SEQ ID NO: 336 - protein, 7 aa, Artificial Sequence
  Synthetic Construct
SDDKRPS

SEQ ID NO: 337 - protein, 5 aa, Artificial Sequence
  Synthetic Construct
GSYSS

SEQ ID NO: 338 - protein, 3 aa, Artificial Sequence
  Synthetic Construct
IYS

SEQ ID NO: 339 - protein, 9 aa, Artificial Sequence
  Synthetic Construct
GGYDQSSYT

SEQ ID NO: 340 - protein, 5 aa, Artificial Sequence
  Synthetic Construct
GDYYS

SEQ ID NO: 341 - protein, 120 aa, Artificial Sequence
  Synthetic Construct
DVQLVESGGGVVRPGESLRLSCAASGFSFSIYAMSWVRQAPGEGLEWVSTIGADDTYYADSVKGRFTISRDNSKNTLYLQMNSLRAEDTAVYYCAKDSTVGWSGDFFDYWGLGTLVTVSS

SEQ ID NO: 342 - protein, 118 aa, Artificial Sequence
  Synthetic Construct
DVQLVESGGAVVRPGESLRLSCAASGFTFSSYAMSWVRQAPGKGLEWLAGISAGGSDTYYIDSVKGRFTISRDNSENSLYLQMNSLTAEDTAVYYCARETWNHLFDYWGLGTLVTVSS

SEQ ID NO: 343 - protein, 107 aa, Artificial Sequence
  Synthetic Construct
ALTQPASVSANPGETVKITCSGGDWYSTYYGWYQQKSPGSAPVTVIHSDDKRPSDIPSRFSGSASGSAATLTITGVRVEDEAVYYCAGYDGRTYINTFGAGTTLTVL

SEQ ID NO: 344 - protein, 119 aa, Artificial Sequence
  Synthetic Construct
DVQLVESGGGVVRPGESLRLSCAASGFTFSSYAMSWVRQAPGKGLEWLAGISAGGSDTYYIDSVKGRFTISRRQFQEQSLSPNEPALTAEDTAVYYCARETWNHLFDYWGLGTLVTVSS

SEQ ID NO: 345 - protein, 107 aa, Artificial Sequence
  Synthetic Construct
ALTQPASVSANPGETVKITCSGGDYYSTYYGWYQQKSPGSAPVTVIHSDDKRPSDIPSRFSGSASGSAATLTIAGVRVEDEAVYFCGAYDGRTYINTFGAGTTLTVL

SEQ ID NO: 346 - protein, 118 aa, Artificial Sequence
  Synthetic Construct
DVQLVESGGGVVRPGESLRLSCAASGFTFSSHAMSWVRQAPGKGLEWLAGISAGGSDTYYIDSVKGRFTISRDNSKSSLYLRMNSLTAEDTAVYYCARETWNHLFDYWGLGTLVTVSS

SEQ ID NO: 347 - protein, 107 aa, Artificial Sequence
  Synthetic Construct
ALTQPASVSANPGETVKITCSGGDYYSTYYAWYQQKSPGSAPVTVIHSDDERPSDIPSRFSGSASGSAATLIITGVRVEDEAVYFCGGYDGRTYINTFGAGTTLTVL

SEQ ID NO: 348 - protein, 118 aa, Artificial Sequence
  Synthetic Construct
DVQLVESGGGVVRPGESLRLSCAASGFTFSSNAMSWVRQAPGKGLEWLAGISAGGSDTYYPASVKGRFTISRDNPKNTLYLQMNTLTAEDTAVYYCARETWNHLFDYWGLGTLVTVSS

SEQ ID NO: 349 - protein, 107 aa, Artificial Sequence
  Synthetic Construct
ALTQPASVSANPGETVKIACSGGSYYSYYYGWYQQKSPGSALVTVIYSDDKRPSGIPSRFSGSASGSTATLTITGVRAEDEAVYYCGGYDYSSYTNDFGAGTTLTVL

SEQ ID NO: 350 - protein, 118 aa, Artificial Sequence
  Synthetic Construct
DVQLVESGGGVVRPGESLRLSCAASGFTFSTYAMSWVRQAPGKGLEWVSGISASGSGTYYGDSVKGRFTMSRDNSKNTLYLQMNSLTAEDTAVYYCARETWNHLFDYWGLGTLVTVSS

SEQ ID NO: 351 - protein, 105 aa, Artificial Sequence
  Synthetic Construct
ALTQPASVSANLGGTVEITCSGGSSSYYGWYQQKSPGSAPVTVIYSDNQRPSDIPSRFSGSASDSTATLTITGVQVEDEAIYYCGGYDSSTYANTFGAGTTLTVL

SEQ ID NO: 352 - protein, 117 aa, Artificial Sequence
  Synthetic Construct
DVQLVESGGGVVRPGESLRLSCAASGFSFSSNAMSWVRQAPGKGLEWVAGISASGDTYYSGSMKGRFTISRDNSKNTLYLQMNSLTAEDTAVYYCARETWNHLFDYWGLGTLVTVSS

SEQ ID NO: 353 - protein, 106 aa, Artificial Sequence
  Synthetic Construct
ALTQPASVSANPGETVKITCSGGSDSYYYGWHQQKSPGSAPVTVIYSDDQRPPDIPSRFSGSASGSTTTLTITGVRAEDEAVYYCGGYDYSTYTNTFGAGTTLTVL

SEQ ID NO: 354 - protein, 117 aa, Artificial Sequence
  Synthetic Construct
DVQLVESGGGVVRPGESLRLSCAVSGFRFSSYAMSWVRQAPGKGLEWVSGISSDSDAYYVDSVKGRFTISRDNSKNTLYLQVNSLTAEDTAVYYCARETWNHLFDYWGLGTMVTVSS

SEQ ID NO: 355 - protein, 107 aa, Artificial Sequence
  Synthetic Construct
ALTQPASVSANLGETVKITCSGGDSSSHYYGWFQQKSPGSAPVTLIYSDDERPSDIPSRFSGSASGSTATLTITGVRVEDEAIYFCGAYDGSTYTNTFGAGTTLTVL

SEQ ID NO: 356 - protein, 117 aa, Artificial Sequence
  Synthetic Construct
DVQLVESGGGVVRPGESLRLSCEASGFTFSSDAMSWVRQAPGKGLEWVSGISSGSSTYYGGSVKGRFTISRDNSKNTLYLQMNSLTAEDTAVYYCARETWNHLFDYWGLGTLVTVSS

SEQ ID NO: 357 - protein, 107 aa, Artificial Sequence
  Synthetic Construct
ALTQPASVSASPGETVEITCSGGSDSSYYYGWYQQKSPGSAPVTVIYSDNKRPSNIPSRFSGSASGSTATLTITGVRVEDEAVYYCGGYDYSTYTNPFGAGTTLTVL

SEQ ID NO: 358 - protein, 117 aa, Artificial Sequence; identical to SEQ ID NO: 139
  Synthetic Construct

SEQ ID NO: 359 - protein, 107 aa, Artificial Sequence
  Synthetic Construct
ALTQPASVSANLGETVEITCSGGDSSSHYYGWYQQKSPGSAPVTVIYSDDERPSDIPSRFSGSASGSTATLTITGVRVEDEAIYYCGAYDGSTYANTFGAGTTLTVL

SEQ ID NO: 360 - protein, 118 aa, Artificial Sequence
  Synthetic Construct
DVQLVESGGGVVRPGESLRLSCAASGFTFSSYAMSWVRQAPGKGLEWLAGISAGGSDTYYIDSVKGRFTISRDNSKNSLYLQVNSLTAEDTAVYYCARETWNHLFDYWGLGTLVTVSS

SEQ ID NO: 361 - protein, 107 aa, Artificial Sequence
  Synthetic Construct
ALTQPASVSANPGETVKITCSGGGYYSTYYGWYQQKSPGSAPVTVIHSDDKRPSDIPSRFSGSASGSAATLTITGVRVEDEAVYYCAGYDGRTYINTFGAGTTLTVL

SEQ ID NO: 362 - protein, 117 aa, Artificial Sequence
  Synthetic Construct
DVQLVESGGGVVRPGESLRLSCAVSGFRFSSHAMSWVRQAPGKGLEWVSGISSGGDTYYVDSVKGRFTISRDNSKNTLYLQVNSLTAEDTAIYYCARETWNHLFDYWGLGTLVTVSS

SEQ ID NO: 363 - protein, 107 aa, Artificial Sequence; identical to SEQ ID NO: 295
  Synthetic Construct

SEQ ID NO: 364 - protein, 118 aa, Artificial Sequence
  Synthetic Construct
DVQLVDSGGGVVRPGESLRLSCAASGFTFSSYAMSWVRQAPGKGLEWLAGISAGGSDTYYIDSVKGRFTISRDNSKNSLYLQMNSLTAEDTAVYYCARETWNHLFDYWGLGTLVTVSS

SEQ ID NO: 365 - protein, 107 aa, Artificial Sequence
  Synthetic Construct
ALTQPASVSANPGETVKITCSGGDYYSTYYGWYQQKSPGSAPVTVIHSDDKRPSDIPSRFSGSASGSAATLTITGVRVEDEAVYFCGAYDGRTYINTFGAGTTLTVL

SEQ ID NO: 366 - protein, 118 aa, Artificial Sequence
  Synthetic Construct
DVQLVESGGGVVRPGESLRLSCAASGFTFSSYAMSWVRQAPGKGLEWLAGISAGGSDTYYIDSVKGRFTISRDNSKNSLYLQMNSLTAEDTAVYYCARETWNHLFDYWGLGTLVTVSS

SEQ ID NO: 367 - protein, 107 aa, Artificial Sequence; identical to SEQ ID NO: 365
  Synthetic Construct

SEQ ID NO: 368 - protein, 118 aa, Artificial Sequence
  Synthetic Construct
DLQLVESGGGVVRPGESLRLSCAASGFTFSSYAMSWVRQAPGKGLEWLAGISAGGSDTYYIDSVKGRFTISRDNSKNSLYLQMNSLTAEDTAVYYCARETWNHLFDYWGLGTLVTVSS

SEQ ID NO: 369 - protein, 107 aa, Artificial Sequence
  Synthetic Construct
ALTQPASVSANPGETVKIICSGGDYYSTYYGWYQQKSPGSAPVTVIHSDDKRPSDIPSRFSGSASGSAATLTITGVRVEDEAVYFCGAYDGRTYINTFGAGTTLTVL

SEQ ID NO: 370 - protein, 118 aa, Artificial Sequence
  Synthetic Construct
DVQLVESGGGVVRPGESLRLSCAASGFTFSSYAMSWVRQAPGKGLEWLAGISAGGSDAYYIDSVKGRFTISRDNSKNSLYLQMNSLTAEDTAVYYCARETWNHLFDYWGLGTLVTVSS

SEQ ID NO: 371 - protein, 107 aa, Artificial Sequence; identical to SEQ ID NO: 343
  Synthetic Construct

SEQ ID NO: 372 - protein, 118 aa, Artificial Sequence; identical to SEQ ID NO: 366
  Synthetic Construct

SEQ ID NO: 373 - protein, 107 aa, Artificial Sequence
  Synthetic Construct
ALTQPASVSANPGETVKITCSGGGYYSTYYGWYQQKSPGSAPVTVIHSDDKRPSDIPSRFSGSASGSAATLTITGVRVEDEAVYYCAGYDARTYINTFGAGTTLTVL

SEQ ID NO: 374 - protein, 117 aa, Artificial Sequence
  Synthetic Construct
DVQLVESGGGVVRPGESLRLSCEASGFTFSSNAMSWARQAPGKGLEWVAGISSGSDTYYGDSVKGRLTISRDNSKNILYLQMNSLTAEDTAVYYCARETWNHLFDYWGLGTLVTVSS

SEQ ID NO: 375 - protein, 107 aa, Artificial Sequence
  Synthetic Construct
ALTQPASVSANPGETVKITCSGGIYSSYYYAWYQQKSPGSAPVTLIYSDDKRPSNIPSRFSGSASGSTATLTITGVRAEDEAVYFCGGYDQSSYTNPFGAGTTLTVL

SEQ ID NO: 376 - protein, 118 aa, Artificial Sequence
  Synthetic Construct
DVQLVESGGGVVRPGESLRLSCAASGFTFSSNAMSWVRQAPGKGLEWLAGISAGDSDTYYPASVKGRFTISRDNPKNTLYLQMNTLTAEDTAVYYCARETWNHLFDYWGLGTLVTVSS

SEQ ID NO: 377 - protein, 107 aa, Artificial Sequence; identical to SEQ ID NO: 349
  Synthetic Construct

SEQ ID NO: 378 - protein, 118 aa, Artificial Sequence; identical to SEQ ID NO: 366
  Synthetic Construct

SEQ ID NO: 379 - protein, 107 aa, Artificial Sequence; identical to SEQ ID NO: 343
  Synthetic Construct

SEQ ID NO: 380 - protein, 118 aa, Artificial Sequence
  Synthetic Construct
DVQLVESGGAVVRPGETLRLSCTASGFTFSSYAMSWVRQAPGKGLEWVSGISASGSDTYYADSVKGRSTISRDNSKNTLYLRMSSLTAEDTAVYYCARETWNHLFDYWGLGTLVTVSS

SEQ ID NO: 381 - protein, 106 aa, Artificial Sequence
  Synthetic Construct
ALTQPASVSANPGETVKITCSGGGTSSYYGWYQQKSPGSAPVTLIHSDDKRPSDIPSRFSGSASGSTATLTITGVQVEDEAVYYCGGYDYTTYVNTFGAGTTLTVL

SEQ ID NO: 382 - protein, 118 aa, Artificial Sequence; identical to SEQ ID NO: 366
  Synthetic Construct

SEQ ID NO: 383 - protein, 107 aa, Artificial Sequence
  Synthetic Construct
ALTQPASVSANPGETVKITCSGGGYYSTYYGWYQQRSPGSAPVTVIHSDDKRPSDIPSRFSGSASGSAATLTITGVRVEDEAVYYCAGYDGRTYLNTFGAGTTLTVL

SEQ ID NO: 384 - protein, 118 aa, Artificial Sequence
  Synthetic Construct
DVQLVESGGAVVRPGETLRLSCTASGFTFSSYAMSWVRQAPGKGLEWVSGISASGSDTYYADSVKGRSTISRDNSKNTLYLRMSSLTAEDTAVYYCARETWNHLFDYWGLGTLVTLSS

SEQ ID NO: 385 - protein, 106 aa, Artificial Sequence
  Synthetic Construct
ALTQPASVSANPGETVKITCSGGGTSSYYGWYQQKSPGSAPVTLIHSDDKRPSDIPSRFSGSASGSTATLTITGVQAEDEAVYYCGGYDYTTYVNTFGAGTTLTVL

SEQ ID NO: 386 - protein, 119 aa, Artificial Sequence
  Synthetic Construct
DVQLVESGGGVVRPGESLRLSCAASGFTFSTSDMNWVRQAPGEGLEWVSLISGSGEITYYADSVKGRFTISRDNSKNTLYLQMNSLRAEDTAVYYCAKENDRYRFFDYWGLGTLVTVSS

SEQ ID NO: 387 - protein, 108 aa, Artificial Sequence
  Synthetic Construct
ETVLTQSPGILSLSPGERATLTCRASQSVYTYLAWYQEKPGQAPRLLIYGASSRAAGIPDRFSGSGSGTEFTLTISSLQSEDFAVYYCQQYYDRPPLTFGGGTKVEIK

SEQ ID NO: 388 - protein, 119 aa, Artificial Sequence
  Synthetic Construct
DVQLVESGGGVVRPGESLRLSCAASGFTFSSYDMNWVRQAPGEGLEWVSLISGSGEIIYYADSVKGRFTISRDNSKNTLYLQMNSLRAEDTAVYYCAKENNRYRFFDYWGLGTLVTVSS

SEQ ID NO: 389 - protein, 108 aa, Artificial Sequence
  Synthetic Construct
KTVLTQSPGTLSLSPGERATLTCRADQSVYTYLAWYQERPGQAPRLLIYDASSRATGIPDRFSGSGSGTEFTLTISSLQSEDFAVYYCQQYYDRPPLTFGGGTKVEIK

SEQ ID NO: 390 - protein, 119 aa, Artificial Sequence; identical to SEQ ID NO: 388
  Synthetic Construct

SEQ ID NO: 391 - protein, 108 aa, Artificial Sequence
  Synthetic Construct
ETVLTQSPGTLTLSPGERATLSCRASQSVYTYLAWYQEKPGQAPRLLIYGASSRATGVPDRFSGSGSGTEFTLTISSLQSEDFAVYYCQQYYDRPPLTFGGGTKVEIK

SEQ ID NO: 392 - protein, 119 aa, Artificial Sequence
  Synthetic Construct
DVQLVESGGGVVRPGESLRLSCAASGFTFSSYDMNWVRQAPGEGLEWVSLISGSGEIIYYADSVKGRFTISRDNSKNTLYLQMNSLRAEDTAVYYCAKENDRYRFFDYWGLGTLVTVSS

SEQ ID NO: 393 - protein, 108 aa, Artificial Sequence; identical to SEQ ID NO: 134
  Synthetic Construct

SEQ ID NO: 394 - protein, 119 aa, Artificial Sequence; identical to SEQ ID NO: 388
  Synthetic Construct

SEQ ID NO: 395 - protein, 108 aa, Artificial Sequence
  Synthetic Construct
ETVLTQSPGTLSLSPGERATLNCRASQSVYTYLAWYQEKPGQAPRLLIYDASSRATGIPDRFSGSGSGTEFTLTISSLESEDFAVYYCQQYYDRPPLTFGGGTKVEIK

SEQ ID NO: 396 - protein, 119 aa, Artificial Sequence; identical to SEQ ID NO: 133
  Synthetic Construct

SEQ ID NO: 397 - protein, 108 aa, Artificial Sequence
  Synthetic Construct
ETVLTQSPGTLSLSPGERATLNCRASQSVYSYLAWYQERPGQAPRLLIYGASTRATGIPDRFSGSGSGTEFTLTISSLESDDFAVYYCQQYYDRPPLTFGGGTKVEIK

SEQ ID NO: 398 - protein, 119 aa, Artificial Sequence
  Synthetic Construct
DVQLVESGGGVVRPGESLRLSCAASGFTFSSSDMNWVRQAPGEGLEWVSLISGSGEITYYADSVKGRFTISRDNSKNTLYLQMNSLRAEDTAIYYCAKENNMYRFFDYWGLGTLVTVSS

SEQ ID NO: 399 - protein, 108 aa, Artificial Sequence
  Synthetic Construct
ETVLTQSPGTLSLSPGERATLSCRASQSVYTYLAWYQQKPGQPPRLLIHAARNRAAGIPDRFSGSGSGTEFTLTISSLQSEDFAVYYCQQYYDRPPLTFGGGTKVEIK

SEQ ID NO: 400 - protein, 119 aa, Artificial Sequence
  Synthetic Construct
DVQLVESGGGVVRPGESLRLSCAASGFTFSSYDMNWVRQAPGEGLEWVSLISGSGEIIYYADSVKGRFTISRDNSKNTLYLQMNSLRAEDTAVYYCAKEDNRYRFFDYWGLGALVTVSS

SEQ ID NO: 401 - protein, 108 aa, Artificial Sequence
  Synthetic Construct
ETVLTQSPGTLTLSPGERTTLTCRASQSVYTYLAWYQEKPGQAPRLLIYGASSRATGIPDRFSGSGSGTEFTLTISSLQSEDFAVYYCQQYYDRPPLTFGGGTKVEIK

SEQ ID NO: 402 - protein, 119 aa, Artificial Sequence
  Synthetic Construct
DVQLVESGGGVVRPGESLRLSCAASGFTFSSYDMNWVRQAPGEGLEWVSLISGSGEITYYADSVKGRFTISRDNSKNTLYLQMNSLRAEDTAVYYCAKENNRYRFFDYWGLGTLVTVSS

SEQ ID NO: 403 - protein, 108 aa, Artificial Sequence
  Synthetic Construct
ETVLTQSPGTLSLSPGERATLSCRASQSVYTYLAWYQEKPGQAPRLLIYAASTRATGIPDRFSGSGSGTEFTLTISSLQSEDFAVYYCQQYYDRPPLTFGGGTKVEIK

SEQ ID NO: 404 - protein, 119 aa, Artificial Sequence
  Synthetic Construct
DVQLVESGGGVVRPGESLRLSCAASGFSFSSYAMNWVRQAPGEGLEWVSRINSGGGGTDYAESVKGRFTISRDNSENTLYLQMNSLRAEDTAVYYCAKQYDWNGFFDYWGLGALVTVSS

SEQ ID NO: 405 - protein, 108 aa, Artificial Sequence
  Synthetic Construct
ETVLTQSPATLSVSPGERATLSCRASQTVGSKLAWHQQKPGQAPRLLIYDATNRATGIPDRFSGSGSGTDFTLTISGLQTEDSAVYYCQQYYYWPPYRFGGGTKVEIK

SEQ ID NO: 406 - protein, 119 aa, Artificial Sequence
  Synthetic Construct
DVQLVESGGGVVRPGESLRLSCAASGFSFSSHAMNWVRQAPGEGLEWVSRINSGGGGTDYAESVKGRFTISRDNSENTLYLQMNSLRAEDTAVYYCAKQYDWNGFFDYWGLGALVTVSS

SEQ ID NO: 407 - protein, 108 aa, Artificial Sequence; identical to SEQ ID NO: 95
  Synthetic Construct

SEQ ID NO: 408 - protein, 117 aa, Artificial Sequence
  Synthetic Construct
DVQLVESGGGLVRPGESLRLSCAASGFTFTNYAVTWVRQAPGEGLEWVSLISVTGTTYYADSVKGRFTISRDNSKSTLYLQMNGLRAEDTAVYYCAKVTWKNVFDYWGLGTLVTVSS

SEQ ID NO: 409 - protein, 108 aa, Artificial Sequence; identical to SEQ ID NO: 291
  Synthetic Construct

SEQ ID NO: 410 - protein, 117 aa, Artificial Sequence; identical to SEQ ID NO: 408
  Synthetic Construct

SEQ ID NO: 411 - protein, 108 aa, Artificial Sequence
  Synthetic Construct
EIVLTQSPGTLSVSPGERATFSCRASQTVGSKLAWYQQKPGQAPRLLIYDANTRATGIPARFSGSRSGTEFTLTISSLQSEDFAVYYCQQHTDWPPYTFGGGTKVEIK

SEQ ID NO: 412 - protein, 118 aa, Artificial Sequence
  Synthetic Construct
DVQLVESGGGVVRPGESLRLSCAASGFTFSDHDMSWVRQGPGEGLEWVAGISLRGGVTWYADSVKGRFTISRDNSKNTLYLRLFSLRTEDTAIYYCARESWNTFFDYWGLGTLVTVSS

SEQ ID NO: 413 - protein, 108 aa, Artificial Sequence; identical to SEQ ID NO: 279
  Synthetic Construct

SEQ ID NO: 414 - protein, 119 aa, Artificial Sequence
  Synthetic Construct
DVQLVESEGGVVRPGESLRLSCEASGFTFRNSYMTWVRQAPGEGLEWVSTISDTGDTAYYADSVKGRFTISRDNSKNSLYLQMNSLRAEDTAIYYCAKSWIWWTFFDYWGLGTLVTVSS

SEQ ID NO: 415 - protein, 103 aa, Artificial Sequence
  Synthetic Construct
ALTQPASVSANLGGTVEITCSGGNSNHYGWYQQKSPGSAPVTLIYADTNRPSNIPSRFSGSTSGSTSTLTITGVQAEDEAVYYCGGSSTGDGIFGAGTTLTVL

SEQ ID NO: 416 - protein, 108 aa, Artificial Sequence
  Synthetic Construct
SYELTQPPSVSVSPGQTARITCSGGAYSSYYYAWYQQKPGQAPVLVIYSDSKRPSGIPERFSGSSSGTTVTLTISGVQAEDEADYYCGGYDQSSYTNPFGGGTKLTVL

SEQ ID NO: 417 - protein, 108 aa, Artificial Sequence
  Synthetic Construct
EIVLTQSPGTLTLSPGERATLSCRASQSVYTYLAWYQQKPGQAPRLLIYGASSRATGIPDRFSGSGSGTEFTLTISSLQSEDFAVYYCQQYYDRPPLTFGGGTKVEIK

SEQ ID NO: 418 - protein, 108 aa, Artificial Sequence
  Synthetic Construct
EIVLTQSPGTLSLSPGERATLTCRASQSVYTYLAWYQQKPGQAPRLLIYGASSRATGIPDRFSGSGSGTEFTLTISSLQSEDFAVYYCQQYYDRPPLTFGGGTKVEIK

SEQ ID NO: 419 - protein, 108 aa, Artificial Sequence
  Synthetic Construct
EIVLTQSPGTLSLSPGERATLSCRASQSVYTYLAWYQEKPGQAPRLLIYGASSRATGIPDRFSGSGSGTEFTLTISSLQSEDFAVYYCQQYYDRPPLTFGGGTKVEIK

SEQ ID NO: 420 - protein, 120 aa, Artificial Sequence
  Synthetic Construct
DVQLLESGGGVVQPGGSLRLSCAASGFSFSNFALTWVRQAPGEGLEWVSTIGSGDTYYADSVKGRFTISRDNSKNTLYLQMNSLRAEDTAVYYCAKDSTVSWSGDFFDYWGLGTLVTVSS

SEQ ID NO: 421 - protein, 120 aa, Artificial Sequence
  Synthetic Construct
DVQLLESGGGVVQPGGSLRLSCAASGFSFSNFAVTWVRQAPGEGLEWVSTIGSGDTYYADSVKGRFTISRDNSKNTLYLQMNSLRAEDTAVYYCAKDSTVSWSGDFFDYWGLGTLVTVSS

SEQ ID NO: 422 - protein, 120 aa, Artificial Sequence
  Synthetic Construct
DVQLVESGGGVVRPGESLRLSCAASGFSFSIYALSWVRQAPGEGLEWVSTIGADDTYYADSVKGRFTISRDNSKNTLYLQMNSLRAEDTAVYYCAKDSTVGWSGDFFDYWGLGTLVTVSS

SEQ ID NO: 423 - protein, 120 aa, Artificial Sequence
  Synthetic Construct
DVQLVESGGGVVRPGESLRLSCAASGFSFSIYAVSWVRQAPGEGLEWVSTIGADDTYYADSVKGRFTISRDNSKNTLYLQMNSLRAEDTAVYYCAKDSTVGWSGDFFDYWGLGTLVTVSS

SEQ ID NO: 424 - protein, 119 aa, Artificial Sequence
  Synthetic Construct
DVQLVESGGGVVRPGESLRLSCAASGFTFSSYDLNWVRQAPGEGLEWVSLISGSGEIIYYADSVKGRFTISRDNSKNTLYLQMNSLRAEDTAVYYCAKENNRYRFFDDWGLGTLVTVSS

SEQ ID NO: 425 - protein, 119 aa, Artificial Sequence
  Synthetic Construct
DVQLVESGGGVVRPGESLRLSCAASGFTFSSYDVNWVRQAPGEGLEWVSLISGSGEIIYYADSVKGRFTISRDNSKNTLYLQMNSLRAEDTAVYYCAKENNRYRFFDDWGLGTLVTVSS

SEQ ID NO: 426 - protein, 106 aa, Artificial Sequence
  Synthetic Construct
GQPKAAPSVTLFPPSSEELQANKATLVCLISDFYPGAVTVAWKADSSPVKAGVETTTPSKQSNNKYAASSYLSLTPEQWKSHRSYSCQVTHEGSTVEKTVAPTECS